European Patent Application EP 4 545 559 A2, published April 30, 2025. Title: ANTI-SARS-COV-2 HUMAN MONOCLONAL ANTIBODY, PHARMACEUTICAL COMPOSITION, DIAGNOSTIC KIT AND USE THEREOF. Applicant: INSTITUTO BUTANTAN. The sequence listing filed with the application follows.

SEQUENCE LISTING (360 sequences)

SEQ ID NO: 1 - protein, 117 aa, synthetic construct
  REGION 1..117: note = heavy chain S.8.1.A4
EVQLVESGGGLVQPGGSLRLSCAASGIIVSNNYMSWVRQAPGKGLEWVSIIYSGGSTFYADSVKGRFTISRDNSKNTLYLQMNSLRVEDTAVYYCARDLGGLRLDYWGQGTLVTVSS

SEQ ID NO: 2 - protein, 107 aa, synthetic construct
  REGION 1..107: note = light chain S.8.1.A4_K
DIQMTQSPSSLSASVGDRVTITCQASQDINICLNWYQQKPEKAPKLLIYDASNLETGVPSRFSGSGSGTDFTFTISSLQPEDIATYYCQQYDNLPQTFGQGTKVEIK

SEQ ID NO: 3 - protein, 117 aa, synthetic construct
  REGION 1..117: note = heavy chain S.9.1.A12
EVQLVESGGGLVQPGGSLRLSCAVSGFIVGRNYMSWVRQAPGKGLEWVSVIYPGGSTFYADSVKGRFTISRDNSKSTLFLQMNSLRAEDTAVYYCARDRGEQFFDYWGQGTLVTVSS

SEQ ID NO: 4 - protein, 107 aa, synthetic construct
  REGION 1..107: note = light chain S.9.1.A12_K
DIQMTQSPSSLSASVGDRVTITCRASQGISNYLAWYQQKPGKAPKLLIYAASTLQSGVPSRFSGSGSGTDFTLTISSLQPEDVATYYCQKYNSAPPTFGGGTKVEIK

SEQ ID NO: 5 - protein, 118 aa, synthetic construct
  REGION 1..118: note = heavy chain S.9.1.B11
  SITE 11: note = misc_feature - Xaa can be any naturally occurring amino acid
EVQLVETGGGXIQPGGSLRLSCAASGITVSRNYMNWVRQAPGKGLEWVSLIYSGGSTFYADSVKGRFTISRDNSKNTLYLQMNSLRAEDTAVYYCARDLADRGGMDVWGQGTTVTVSS

SEQ ID NO: 6 - protein, 108 aa, synthetic construct
  REGION 1..108: note = light chain S.9.1.B11_L
SYELTQPPSVSVAPGKTARITCGGNNVGSQSVHWYQQRSGQAPVLVVYDDGDRPSGIPGRFSGSNSGNTATLTISRVEAGDEADYFCQAWDSSRDHVVFGGGTKLTVL

SEQ ID NO: 7 - protein, 120 aa, synthetic construct
  REGION 1..120: note = heavy chain S.9.1.C10
QVQLVQSGAEVKKPGASVKISCKASGYTFIHYYMHWVRQAPGQGLEWMGIINPSGGGTTYTQKFQGRVTMTRDTSTSTVYMELSSLRSEDTAVYYCARDLAGYTSEFDYWGQGTLVTVSS

SEQ ID NO: 8 - protein, 107 aa, synthetic construct
  REGION 1..107: note = light chain S.9.1.C10_K
IQMTQSPSSLSASVGDRVTITCRASQGIRNDLGWYQQKPGKAPKRLIYAASSLQSGVPSRFSGSGSGTEFTLTISSLQPEDVATYYCLQHNSYPMCSFGQGTKLEIK

SEQ ID NO: 9 - protein, 128 aa, synthetic construct
  REGION 1..128: note = heavy chain S.9.1.C9
QVQLVESGGGVVQPGRSLGLSCAVSGFTFSNYGMDWVRQAPGKGLEWVAVTSYDGSNKYYADSVKGRFTISRDNSKNTLYLQMNSLRTEDTAVYYCAKHGGGPYCGGGTCYLAYFDYWGQGTLVTVSS

SEQ ID NO: 10 - protein, 109 aa, synthetic construct
  REGION 1..109: note = light chain S.9.1.C9_K
DIQMTQSPSSLSASVRDRVTITCQASQDISKFLNWYQQKPGKAPKLLIYDASNLETGVPSRFSGSGSGTDFTFTISSLQPEDIATYYCQQYDNLPITFGQGTRLEIKRT

SEQ ID NO: 11 - protein, 123 aa, synthetic construct
  REGION 1..123: note = heavy chain S.9.1.H5
QVQLVESGGGVVQPGRSLRLSCAASGFTFSRYGMHWVRQAPGKGLEWVALISYDGTNKYYADSVKGRFTISRDNSKSTQYLQMNSLRAEDTAVYFCAKESFGYASGSYYFDYWGQGTLVTVSS

SEQ ID NO: 12 - protein, 107 aa, synthetic construct
  REGION 1..107: note = light chain S.9.1.H5_K
DIQMTQSPSSLSASVGDRITITCQASQDISNYLNWYQQKPGKAPKLMIYDASNLETGVPSRFSGSGAGTDFTFTISSLQPEDFARYYCQQYGNLPLTFGGGTKVEIK

SEQ ID NO: 13 - protein, 118 aa, synthetic construct
  REGION 1..118: note = heavy chain S.9.2.B8
EVQLVETGGGLIQPGGSLRLSCAASGLIVSSNYMTWVRQAPGKGLEWVSVLYSGGTTYYADSVKGRVTISRDNSKNTLYLQVNSLTVADTAVYYCARDLADRGGMDVWGQGTTVTVSS

SEQ ID NO: 14 - protein, 108 aa, synthetic construct
  REGION 1..108: note = light chain S.9.2.B8_L
SYELTQPPSVSVAPGQTARITCGGNNIGSQSVHWYQQKPGQAPVLVVYDDSDRPSGIPERFSGSKSGNMATLTISRVEAGDEADYYCQVWDSSSDHVVFGGGTKLTVL

SEQ ID NO: 15 - protein, 117 aa, synthetic construct
  REGION 1..117: note = heavy chain S.9.2.D3
EVQLVESGGGLVQPGGSLRLSCAASEFIVSSNYMSWVRQAPGKGLEWVSVIYSGGSTFYADSVKGRFTISRDNSKNTLYLQMDALRAEDTAVYYCARDYGEFYFDYWGQGTLVTVSS

SEQ ID NO: 16 - protein, 108 aa, synthetic construct
  REGION 1..108: note = light chain S.9.2.D3_K
EIVLTQSPGTLSLSPGERATLSCRASQSVSNSYLAWYQQKPGQAPRLLIYGASSRATGIPDRFSGSGSGTDFTLTISRLEPEDFAVYYCQQYDSSPRTFGQGTKVEIK

SEQ ID NO: 17 - protein, 125 aa, synthetic construct
  REGION 1..125: note = heavy chain S.9.2.D7
EVQLLESGGGLIQTGGSLRLSCAASGFTFSSYAMSWVRQAPGKGLEWVSVISDSGGSTYYADSVKGRLTISRDNSKNTLYVQMNSLRAEDTAVYYCAKGKGGIAAAGPAFLFDYWGQGTLVTVSS

SEQ ID NO: 18 - protein, 107 aa, synthetic construct
  REGION 1..107: note = light chain S.9.2.D7_K
DIQMTQSPSLLSASAGDRVTISCRMSQGISSYLAWYQQKPGKAPELLISSASTLQSGVPSRFSGSGSGTDFTLTISYLQSEDFATYYCQQYYSFPTTFGGGTKVEIK

SEQ ID NO: 19 - protein, 120 aa, synthetic construct
  REGION 1..120: note = heavy chain S.9.2.E9
QVQLVQSGAEVKKPGASVKVSCQASGYSFTYYYMHWVRQAPGQGLEWMGIINPSGGGTSYAQKFQGRVTMTRDTSTSTVYMELSSLRSEDTAVYYCARDLAGVTSEFDYWGQGTLVTVSS

SEQ ID NO: 20 - protein, 107 aa, synthetic construct
  REGION 1..107: note = light chain S.9.2.E9_K
IQMTQSPSSLSASVGDRVTITCRASQDIRHDLGWYQQKPGKAPKRLIYAASSLHSGVPSRFSGSGSGTEFTLTISSLQPEDFATYYCLQHNSYPMCSFGQGTKLEIK

SEQ ID NO: 21 - protein, 123 aa, synthetic construct
  REGION 1..123: note = heavy chain S.9.2.F4
QVQLVESGGGVVQPGRSLRLSCAASGFTFSSYGIHWVRQAPGKGLEWVAVIANDGSNKYYRDSVKGRFTISRDNSKNTLYLQMNSLRVEDTAVYYCAKGLAGIAAAGTPFDYWGQGTLVTVSS

SEQ ID NO: 22 - protein, 107 aa, synthetic construct
  REGION 1..107: note = light chain S.9.2.F4_K
EIVLTQSPYLLSASTGDRVTISCRMTQGISSFLAWYQQKPGKAPELLIYAASTLQSGVPSRFSGSGSGTDFTLTISSLQPEDFATYYCQQYYSFPPTFGQGTKLEIK

SEQ ID NO: 23 - protein, 117 aa, synthetic construct
  REGION 1..117: note = heavy chain S.9.3.B2
EVQLVESGGGLVQPGGSLRLSCAASGLTVSSNYMSWVRQAPGKGLEWVSIIYSGGSTFYADSVKGRFTISRHNSKNTLYLQMNSLRAEDTAVYYCARDLVYYGMDVWGQGTTVTVSS

SEQ ID NO: 24 - protein, 108 aa, synthetic construct
  REGION 1..108: note = light chain S.9.3.B2_K
DIQLTQSPSFLSASVGDRVTITCRASQGISNYLAWYQQKPGKAPKLLIYAASTLQSGVPSRFSGSGSGTEFTLTISSLQPEDFATYYCQQLDSYPPLIFGGGTKVEIK

SEQ ID NO: 25 - protein, 117 aa, synthetic construct
  REGION 1..117: note = heavy chain S.9.3.G2
EVQLVESGGGLVRPGGSLRLSCAASGIIVSRNYMSWVRQAPGKGLEWVSVIYSGGSTFYADSVKGRFTISRDNSKNTLYLQMNGLRAEDTAVYYCARDLSYYGMDVWGQGTTVTVSS

SEQ ID NO: 26 - protein, 107 aa, synthetic construct
  REGION 1..107: note = light chain S.9.3.G2_K
DIQLTQSPSFLSASVGDRVTITCRASQGISSYLAWYQQKPGKAPKLLIYAASTLQSGVPSRFSGSGSGTEFTLTISSLQPEDFATYYCQQLNSYPCSFGQGTKLEIK

SEQ ID NO: 27 - protein, 130 aa, synthetic construct
  REGION 1..130: note = heavy chain S.9.4.C7
QVQLVESGGGVVQPGRSLRLSCAASGFTFRNYAMHWVRQAPGKGLEWVTVISYDGSDKYYADSVKGRFTISRDNSKNTLYLQMNSLRAEDTAVYYCAKDPVGGYCSGGRCYFHSHYFDYWGQGTLVTVSS

SEQ ID NO: 28 - protein, 111 aa, synthetic construct
  REGION 1..111: note = light chain S.9.4.C7_L
NFMLTQPHSVSESPGKTVTISCTRSSGSIASYYVQWYQQRPGSSPTTVISEDNQRPSGVPDRFSGSIDSSSNSASLTISGLKTEDEADYYCQSYDSNNHVIFGGGTKLTVL

SEQ ID NO: 29 - protein, 127 aa, synthetic construct
  REGION 1..127: note = heavy chain S.9.4.F4
QVQLVESGGGVVQPGRSLRLSCAASGFTFSHYGMHWVRQAPGKGLEWVAVILYDGSNEYYADSVKGRFTISRDNSKNTLYLQMNSLRAEDTAVYYCAKGAGTYCSGGNCYVAYFDYWGQGTLVTVSS

SEQ ID NO: 30 - protein, 107 aa, synthetic construct
  REGION 1..107: note = light chain S.9.4.F4_K
AIRMTQSPSSLSASVGDRVTITCQASQDISNYLNWYQQKPGKAPKLLIYDASNLETGVPSRFSGSGSGTDFTVTISSLQPEDFATYYCQQYDNLPLTFGGGTKVEIK

SEQ ID NO: 31 - protein, 127 aa, synthetic construct
  REGION 1..127: note = heavy chain S.9.4.H8
  SITE 9: note = misc_feature - Xaa can be any naturally occurring amino acid
QVQLVESGXGVVQPGRSLRLSCAASGFTFSTYGMHWVRQAPGKGLEWVAVISYDGSNKKFADSVKGRFTISRDTSKNTLYLQMNSLRADDTAVYYCAKGAGTYCSAGNCYVAYFDYWGQGTLVTVSS

SEQ ID NO: 32 - protein, 108 aa, synthetic construct
  REGION 1..108: note = light chain S.9.4.E3_K
  SITE 11: note = misc_feature - Xaa can be any naturally occurring amino acid
  SITE 14: note = misc_feature - Xaa can be any naturally occurring amino acid
  SITE 17: note = misc_feature - Xaa can be any naturally occurring amino acid
DIQMTQSPSSXSAXVGXRVTITCQASQDINNYLNWYQQKPGKAPKLLIYDASNLETGVPSRFSGSGSGTDFTFTISSLKPEDIATYYCQQYYSLPPVTFGQGTRLEIK

SEQ ID NO: 33 - protein, 117 aa, synthetic construct
  REGION 1..117: note = heavy chain S.9.5.A9
EVQLVESGGGLVQPGGSLRLSCAASGITVSSNYMSWVRQAPGKGLEWVSVIYSGGSTFYADSVKGRFTISRHNSKNTLYLQMNSLRPEDTAVYYCARDLGENAFDIWGQGTMVTVSS

SEQ ID NO: 34 - protein, 108 aa, synthetic construct
  REGION 1..108: note = light chain S.9.5.A9_K
DIQLTQSPSFLSASVGDRVTITCRASQGISSYLAWYQQKPGKAPKLLIYAASTLQSGVPSRFSGSGSGTEFTLTISSLQPEDFATYYCQQLNSYPGFTFGPGTKVDIK

SEQ ID NO: 35 - protein, 120 aa, synthetic construct
  REGION 1..120: note = heavy chain S.10.1.C6
QLQLQESGPGLVKPSETLSLTCTVSGGSISSSSYYWGWIRQPPGKGLEWIGSFYYSGGSYYNPSLKSRVTISVDTSKNQFSLKLSSVTAADTAVYYCARDEHGDYAVGYWGQGTLVTVSS

SEQ ID NO: 36 - protein, 112 aa, synthetic construct
  REGION 1..112: note = light chain S.10.1.C6_L
QSVLTQPPSVSGAPGQRVTISCTGSSSNIGAGYDVHWYQQLPGTAPKLLIYGNNNRPSGVPDRFSGSKSGTSASLAITGLQAEDEADYYCQSYDSSLSALYVFGTGTKVTVL

SEQ ID NO: 37 - protein, 118 aa, synthetic construct
  REGION 1..118: note = heavy chain S.10.1.D8
  SITE 11: note = misc_feature - Xaa can be any naturally occurring amino acid
EVQLVESGGGXVQPGGSLRLSCAASGLTVSSNYMSWVRQAPGKGLEWVSLIYSGGSTYYADSVKGRFTISRDNSKNTLYLQMNSLRAEDTAVYYCARDVLHRSGMDVWGQGTTVTVSS

SEQ ID NO: 38 - protein, 107 aa, synthetic construct
  REGION 1..107: note = light chain S.10.1.D8_K
  SITE 11: note = misc_feature - Xaa can be any naturally occurring amino acid
DIQMTQSPSSXSASVGDRVTITCQASQDISNYLNWYQQKPGKAPKLLIYDASNLETGVPSRFSGSGSGTDFTFTISSLQPEDIATYYCQQYDNLPRTFGQGTKVEIK

SEQ ID NO: 39 - protein, 118 aa, synthetic construct
  REGION 1..118: note = heavy chain S.10.2.D2
  SITE 16: note = misc_feature - Xaa can be any naturally occurring amino acid
EVQLVESGGGLVQPGXSLRLSCAASGVTVSSNYMSWVRQAPGKGLEWVSVIYSGGSTYYADSVKGRFTISRDNSKNTLHLQMNSLRAEDTAVYYCARDLGPRGAFDIWGQGTMVTVSS

SEQ ID NO: 40 - protein, 108 aa, synthetic construct
  REGION 1..108: note = light chain S.10.2.D2_K
  SITE 11: note = misc_feature - Xaa can be any naturally occurring amino acid
  SITE 13: note = misc_feature - Xaa can be any naturally occurring amino acid
EIVLTQSPGTXSXSPGERATLSCRASQSVSSTYLAWYQQKPGQAPRLLIYGASSRATGIPDRFSGSGSGTDFTLTISRLEPEDFAVYYCQQYGSSPYSFGQGTKLEIK

SEQ ID NO: 41 - protein, 123 aa, synthetic construct
  REGION 1..123: note = heavy chain S.11.2.A5
  SITE 9: note = misc_feature - Xaa can be any naturally occurring amino acid
QVQLVESGXGVVQPGRSLRLTCAASGFPFSTYVMNWVRQAPGKGLEWVASISNDGTRKDYAGSVKGRFSISRDNFNSDLFLQMNTLKTEDTALYWCARTSGRGSRDRGRFDLWGQGTLVTVSS

SEQ ID NO: 42 - protein, 111 aa, synthetic construct
  REGION 1..111: note = light chain S.11.2.A5_K
DIVMTQSPLSLPVTPGEPASISCRSSQSLLDSNGYNYLDWYLQKPGQSPQLLIYLGSNRASGVPDRFSGSGSGTDFTLKISRVEVEDVGVYYCMQSLQGFTFGPGTKVDIK

SEQ ID NO: 43 - protein, 126 aa, synthetic construct
  REGION 1..126: note = heavy chain S.11.2.C5
QVQLVQSGPEVKKPGSSVKVSCKGSEGTFNVYAISWLRQAPGQGLEWMGGIIPMHGKANLAQKFQGRVTIAADGNTNTGYMELSGLRSEDTAIYFCARDYRYCDSSTCYDFAFDIWGQGTMVTVSS

SEQ ID NO: 44 - protein, 106 aa, synthetic construct
  REGION 1..106: note = light chain S.11.2.C5_K
DIQMTQSPSSLSASVGDRVTMSCRASQNISTFLNWYQQEPGKAPKLLIYAASSLQSGVPSRFSGSGSGTDFSLTIRSLQPEDFATYYCQQSYRSKSFGQGTKLEIK

SEQ ID NO: 45 - protein, 127 aa, synthetic construct
  REGION 1..127: note = heavy chain S.11.3.A5
QVQLVQSGAEVKKPGSSMKVSCKTSGGTFNTYATNWVRQAPGQGLEWMGAIIPIFGTTNYAQKFQGRVTITADQSTTTSYMYLNSLTSEDTAVYYCARGTPVWGSSGPLGYNGMDVWGQGTTVTVSS

SEQ ID NO: 46 - protein, 108 aa, synthetic construct
  REGION 1..108: note = light chain S.11.3.A5_K
DIQMTQSPSSLSASVGDRVTITCRASQSISTYLNWYQQKPGKAPRLVIYGASTLHSGVPSRFSGSGSGTAFTLTISNLQPDDFASYYCQQSSSSLALTFGGGTKVEIK

SEQ ID NO: 47 - protein, 132 aa, synthetic construct
  REGION 1..132: note = heavy chain S.11.3.H5
QVQLVQSGAEVRKPGASVEISCKASGYTFTNFYIHWVRQAAGQGLEWMGLINPSGASTTYAPKFQGRITMTRDTSTPTVYMELSSLRSDDTAVYFCARDFSPSVHYCGGDCNSPQYNWFDPWGQGTLVTVSS

SEQ ID NO: 48 - protein, 107 aa, synthetic construct
  REGION 1..107: note = light chain S.11.3.H5_K
EIVLTQSPATLSVSPGERVTLSCRASQIISRYLAWYQQKPGQAPRLLIYGASSRAAGVPVRFSGSGSGTDFTLTISSLQSEDFAVYFCQQYNNWPLTFGGGTKVEIK

SEQ ID NO: 49 - protein, 117 aa, synthetic construct
  REGION 1..117: note = heavy chain S.11.4.F9
EVQLVESGGGLIQPGGSLRLSCVVSGLTVSSNYMSWVRQAPGKGLEWVSVIYSGGSTFYANSVKGRFTISRDNSKNTLYLQMNSLRAEDTAIYYCTRDYGDFYMDVWGKGTTVTVSS

SEQ ID NO: 50 - protein, 107 aa, synthetic construct
  REGION 1..107: note = light chain S.11.4.F9_K
EIVLTQSPGTLSLSPGERATLSCRASQSVISSYLAWYQQKPGQAPRLLIHGASSRATGIPDRFSGSGSGTDFTLTIRRLEPEDFAVYYCQHYGSSRTFGQGTKVEIK

SEQ ID NO: 51 - protein, 120 aa, synthetic construct
  REGION 1..120: note = heavy chain S.1.1.D10
EVQLLESGGGLVQPGGSLRLSCAVSGFTFSSYAMNWVRQAPGKGLEWVSAISGSGDSTYYADSVKGRFTISRDSSKNTLYLQMSSLRAGDTAVYYCAKDTMGHSSLFDYWGQGALVTVSS

SEQ ID NO: 52 - protein, 108 aa, synthetic construct
  REGION 1..108: note = light chain S.1.1.D10_K
EIVMTQSPVSLSVSPGERATLSCRARESVSNNVAWYQQKPGQAPRLLIYGVSTRATGIPARFSGSGSGTEFTLTISSLQSEDFAVYYCQHYNNWPSWTFGQGTKVEIK

SEQ ID NO: 53 - protein, 123 aa, synthetic construct
  REGION 1..123: note = heavy chain S.11.1.C7
QVQLVQSGAEVKKPGASVRVSCKASGYIFSSYYIHWVRQAPGQGLEWMGVIYPSGGSTDYAQIFQGRVTMTRDTSTNTVYMELSGLRSEDTAVYYCARDGKDIVGATLPGRYWGQGTLVTVSS

SEQ ID NO: 54 - protein, 113 aa, synthetic construct
  REGION 1..113: note = light chain S.11.1.C7_K
DIVMTQSPDSLAVSLGERATIYCKSSQSVLNSSNKKNYLAWYQQKPGQPPRLLIYWASTRESGVPDRFSGSGSGTDFTLTITSLQAEDVAVYYCQHYYSPPITFGQGTRLEIK

SEQ ID NO: 55 - protein, 120 aa, synthetic construct
  REGION 1..120: note = heavy chain S.11.1.C8
QVQLVESGGGVVQPGRSLRLSCAASGFTFSTFSMHWVRQAPGKGLEWVAVILYDGTYKSYADSVKGRFTISRDNSGNTLFLQMNSLRAEDSAVYYCARDFGEMTTYFDFWGQGTLVTVSS

SEQ ID NO: 56 - protein, 108 aa, synthetic construct
  REGION 1..108: note = light chain S.11.1.C8_K
DIQMTQPPSSLSASVGDRVTITCRASQSIGNNLNWYQQKPGKAPKLLIYVASSLQSGVPSRFSGSGSGTDFTLTISSLQPEDFATYFCQQSYSTPPWTFGQGTKVEIK

SEQ ID NO: 57 - protein, 126 aa, synthetic construct
  REGION 1..126: note = heavy chain S.11.1.D12
EVQLLESGGGLVQPGGSLRLSCAASGFPFITYPMSWVRQAPGKGLEWVSDIGGIGGSTSYADSVKGRFTISRDNYQNTVYLQMHSLRAEDTAVYYCAKWKSRVDSSYKGGGWFDSWGPGTLVTVSS

SEQ ID NO: 58 - protein, 114 aa, synthetic construct
  REGION 1..114: note = light chain S.11.1.D12_K
DIVMTQSPDSLAVSLGERATIHCKSSQTVVYGSNNKNYLAWYQQKPGQPPKLLIYWASTRESGVPDRFSGSGSGTDFTLTISSLQAEDVAVYYCQQYYGPPPWTFGQGTKVEIK

SEQ ID NO: 59 - protein, 121 aa, synthetic construct
  REGION 1..121: note = heavy chain S.11.1.F4
QVQLVQSGAEVKKPGSSVRVSCKASAGTFSSYAIRWVRQAPGQGLEWMGTIIPIFGTTNYAQKFQGRVSITADESTNTAYMELSSLRSEDTAVYYCARDLETSPLYGLDVWGQGTTVTVSS

SEQ ID NO: 60 - protein, 107 aa, synthetic construct
  REGION 1..107: note = light chain S.11.1.F4_K
DIQMTQSPSSLSASVGDRVTITCRASQTISRYLNWYQQKPGKPPKLLIFAASTLHSGVPSRFSGSGSGTEFTLTITSLHPDDFSTYYCQQTYSSPHTFGQGTKLEIK

SEQ ID NO: 61 - protein, 123 aa, synthetic construct
  REGION 1..123: note = heavy chain S.11.1.H1
QVQLVESGGGVVQPGRSLTLSCSASGFPFSTYVMHWVRQAPGKGLEWVAVISSDGSNENYADSVKGRFTVSRDNFGSTLFLQMSTLRPDDTAVYYCARTAGRGYADRGRLDTWGQGTLVTVSS

SEQ ID NO: 62 - protein, 111 aa, synthetic construct
  REGION 1..111: note = light chain S.11.1.H1_K
DIVMTQSPLYLPVTPGEPASISCRSSQSLLHSNGYNYLDWYLQKPGQSPQLLIYLGSNRASGVPDRFSGSGSGTDFTLKISRVEAEDVGVYYCMQTLQTFTFGPGTKVDIK

SEQ ID NO: 63 - protein, 117 aa, synthetic construct
  REGION 1..117: note = heavy chain S.11.1.H5
EVQLVESAGGLVQPGGSLRLSCSASGFTFSSSPMHWVRQAPGKGLQYVSAVSSAGLTTYYADSVKGRFTISRDNSKNTVFLQMSSLRADDTAVYYCVKGWVGTFDPWGQGTLVTVSS

SEQ ID NO: 64 - protein, 108 aa, synthetic construct
  REGION 1..108: note = light chain S.11.1.H5_K
EIVLTQSPATLSVSPGERATLSCRASQSVSSNLAWYQQKPGQAPRLLIYGASTRATGIPARFSGSGSGTEFTLTISSLQSEDFAVYYCQQYNNWPPYTFGQGTKLEIK

SEQ ID NO: 65 - protein, 123 aa, synthetic construct
  REGION 1..123: note = heavy chain S.11.1.H8
QVQLQESGPGQVKPSQTLSLSCTVSGDSINSVGYYWNWIRQHPGKGLEWIGNIYFYGSTYYNPSLQSRVIISLDTSKNQFSLRLTSVTAADAAVYYCARSYTGYESDDALDIWGQGTMVTVSS

SEQ ID NO: 66 - protein, 106 aa, synthetic construct
  REGION 1..106: note = light chain S.11.1.H8_K
IQMTQSPSSLSASVGDRVTITCRASQDIGSDLGWFQQRPGKAPKRLIYGASSLQSGVPSRVSGSGSGTEFTLTISSLQPEDFASYYCLQYNSYPLTFGGGTKVEIK

SEQ ID NO: 67 - protein, 125 aa, synthetic construct
  REGION 1..125: note = heavy chain S.11.2.A3
EVQLVESGGGLVKPGGSLSLSCAASGLTFSNVWMNWVRQAPGKGLEWVGLIKSATDGGTPYYAAPVKGRFIIPRDDSKNTLYLQMNSLKTEDTAVYFCTTEAPGYSYGYEDFDYWGQGTLVTVSS

SEQ ID NO: 68 - protein, 107 aa, synthetic construct
  REGION 1..107: note = light chain S.11.2.A3_K
EIVLTQSPGTLSLSPGERATLSCRASQNIGMSYVAWYQQKGGQAPRLLIYGVSSRATGIPDRFSGSGSGTDFTLTISRLEPKDSAVYYCQQYGSSHRTFGQGTKLEI

SEQ ID NO: 69 - protein, 127 aa, synthetic construct
  REGION 1..127: note = heavy chain S.2.2.F11
QVQLVQSGAEVKKPGASVKVSCKASGGTSSSYVISWVRQAPGQGLEWMGWINPNSGGANCAQKFQGRVTVTRDTSTSTVYMELSSLRSEDTAVYYCARGPPQGVWFGVSGMDVWGQGNHGHRLLSVD

SEQ ID NO: 70 - protein, 106 aa, synthetic construct
  REGION 1..106: note = light chain S.2.2.F11_K
DIQMTQSPSSLSASVGDRVTITCQASQDISNYLNWYQQKPGKAPKLLIYDASNLETGVPSRFSGSGSGTDFTFTISSLQPEDIATYYCQQYDNLLTFGGGTKVEIK

SEQ ID NO: 71 - protein, 125 aa, synthetic construct
  REGION 1..125: note = heavy chain S.2.2.G8
QVQLVQSEAEVKKPGSSVKVSCRASGGTFNNYAISWVRQAPGQGLEWMGGIFPFRNTAKYAQHFQGRVTITADESTGTAYMELSSLRSEDTAIYYCARGDTIFGVTMGYYAMDVWGQGTTVTVSS

SEQ ID NO: 72 - protein, 108 aa, synthetic construct
  REGION 1..108: note = light chain S.2.2.G8_K
EIVLTQSPVSLSVSPGERATLSCRARESVSNNVAWYQQKPGQAPRLLIYGVSTRATGIPARFSGSGSGTEFTLTISSLQSEDFAVYYCQHYNNWPSWTFGQGTKVEIK

SEQ ID NO: 73 - protein, 125 aa, synthetic construct
  REGION 1..125: note = heavy chain S.2.3.C4
QVQLVRSGAEVKKPGASVKVSCKASGYSFTNYAISWVRQAPGQGLEWMGWISTYNGNPKYAQKLQGRVTMTTDTSTSTAYMDLRSLRSDDTAVYYCARLPFYFYDSSGYDAFDIWGQGTMVTVSS

SEQ ID NO: 74 - protein, 106 aa, synthetic construct
  REGION 1..106: note = light chain S.2.3.C4_K
IQMTQSPSAVSASVGDRVTITCRASQGISDYLVWFQQKPGKVPKRLIYGASSLQSGVPSRFSGSGSGTEFTLTISSLQPEDFATYYCLQHKSYPYTFGQGTKLEIK

SEQ ID NO: 75 - protein, 131 aa, synthetic construct
  REGION 1..131: note = heavy chain S.2.3.G7
QVQLVESGGGLVKPGGSLRLSCAASGFTFSDYYMSWVRQAPGKGLEWVPYISSSGSSINYADSVKGRFTISRDNAKNSLYLQMNNLRAEDTAVYYCARDPGPYYASGSYTTFYYRYGMDVWGQGTTVTVSS

SEQ ID NO: 76 - protein, 108 aa, synthetic construct
  REGION 1..108: note = light chain S.2.3.G7_K
EIVLTQSPATLSLSPGERATLSCRASQSVSSYLAWYQHKPGQAPRLLIYDASNRATGIPARFSGSGSGTDFTLTISSLEPEDFAVYYCQQRSNWPPLTFGGGTKVEIK

SEQ ID NO: 77 - protein, 122 aa, synthetic construct
  REGION 1..122: note = heavy chain S.2.4.D2
QVQLVESGGGVVQPGGSLRLSCAASGFTFSSYAMHWVRQAPGKGLEWVAYIQYDGTNKFYADSVKGRFTISRDNSKNTLYLQMNSLRVEDSAVFYCAKSRGSGSYSFFFHHWGQGTLVTVSS

SEQ ID NO: 78 - protein, 107 aa, synthetic construct
  REGION 1..107: note = light chain S.2.4.D2_K
DIQMTQSPFSLSASVGDRVTITCRASPGISNYLAWYQQKPGKVPKLLIYAASTLQSGVPSRFSGSGSGTDFTLTITSLQPEDVATYYCQKYNNAPFTFGPGTKVDIK

SEQ ID NO: 79 - protein, 132 aa, synthetic construct
  REGION 1..132: note = heavy chain S.2.4.E3
EVQLLESGGDLVQPGGSLRLSCTASGFTFSSYAMSWVRQAPGKGLEWVSRISGSGSGTFYRDSVKGRFTVSRDNPNNTLFLQMNSLRAEDTAVYYCAKDGPYYDILTGPGHPSYYYYGMDVWGQGTTVTVSS

SEQ ID NO: 80 - protein, 106 aa, synthetic construct
  REGION 1..106: note = light chain S.2.4.E3_K
IQMTQSPSSVSASVGDRVTITCRASQHVSSSLVWYQQKPGRAPRLLIFAASKLQSGVSSRFSGSGSGTDFTLTISSLQPEDFATYYCQQANSFPYTFGQGTKLEIK

SEQ ID NO: 81 - protein, 121 aa, synthetic construct
  REGION 1..121: note = heavy chain S.2.4.E8
EVQLVESGGVVVQPGGSLRVSCAASGFTFDDYAMHWVRQAPGRGLEWVSVISWDASSTYYADSVKGRFTISRDNSKHSLFLQMNSLRPEDTAFYFCAKDMTPYGSGSPDYWGQGTLVTVSS

SEQ ID NO: 82 - protein, 108 aa, synthetic construct
  REGION 1..108: note = light chain S.2.4.E8_K
DIQMTQSPSSLSASVGDRVVITCRASQSISGYLNWYQQKPGKAPKLLIHGTSSLQSGVPSRFSGSGAGTDFTLTISSLQPEDFATYFCQQSYSAPLWTFGQGTKVEIK

SEQ ID NO: 83 - protein, 125 aa, synthetic construct
  REGION 1..125: note = heavy chain S.3.1.B7
QVQLVESGGGVVQPGGSLRLSCAASGFTFRNYALHWVRHTPGKGLEWVAVIWYDENSKYYAESVEGRFTVSRDNSKNTLFLQMNNLRAADAGVYYCARDPGSTSDSSGYYGIDFWGQGTLVTVSS

SEQ ID NO: 84 - protein, 112 aa, synthetic construct
  REGION 1..112: note = light chain S.3.1.B7_K
DVVMTQSPLSLPVTLGQPASISCRSSQSLVYSDGNTYLNWFHQRPGQSPRRLIYRVSKRDSGVPDRFSGSGSGNDFTLKISRVEAEDVGVYYCMQGTHWPLTFGGGTKVEIK

SEQ ID NO: 85 - protein, 117 aa, synthetic construct
  REGION 1..117: note = heavy chain S.3.1.E2
QVQLQESGPGLVKPSETLSLTCTVSGGSITSDHWTWIRQPPGKGLEWIAYMEHNGSPTYNPSVRSPVAMSLDTSKNQLSLKVYSVTAADSAVYYCARAATSSAIDSWGQGTLVTVSS

SEQ ID NO: 86 - protein, 106 aa, synthetic construct
  REGION 1..106: note = light chain S.3.1.E2_K
  SITE 9: note = misc_feature - Xaa can be any naturally occurring amino acid
  SITE 11: note = misc_feature - Xaa can be any naturally occurring amino acid
DIQMTQSPXTXSASVGDRVTITCRASQSISGGLAWYQQKAGKAPKLLIYKASSLESGVPSRFSGSASGTEFTLTISSLQPDDFATYYCHQYNERWTFGQGTKVEIK

SEQ ID NO: 87 - protein, 127 aa, synthetic construct
  REGION 1..127: note = heavy chain S.3.1.G5
RCTSSQLQQWGAGLLKPSETLSLTCSVYGESFSGYYWNWIRQPPGKRLEWIGEINHSGSANYNPSLKSRVSILVDTSRHQIFLRLSSVTAADTAVYYCARAYGSGSYTWGWAPFDYWGQGSLVTVSS

SEQ ID NO: 88 - protein, 108 aa, synthetic construct
  REGION 1..108: note = light chain S.3.1.G5_K
DIQLTQSPGTLSLSPGERATLSCRASQSISSTFLAWYQQIPGQAPRLLIYGASSRAIGIPDRFSGSGSGTDFTLTISRLEPQDFAVYYCQQYGRSPHTFGQGTKLEIK

SEQ ID NO: 89 - protein, 129 aa, synthetic construct
  REGION 1..129: note = heavy chain S.3.2.C7
QVQLVESGGALVKPGESLRLSCVGSGFTFSDFYMSWIRQAPGKGLEWVSAISSSGSNIYHGDSLKGRFTISRDNAKNSMYLQMNSLRAEDTAVYYCARFLNRYYGSGSYGYYYHAVDVWGQGTTVTVSS

SEQ ID NO: 90 - protein, 117 aa, synthetic construct
  REGION 1..117: note = light chain S.3.2.C7_L
TGSWAQSALTQPASVSGSPGQSITIPCTGTSSDVGGHNYVSWYQHHPGKVPQLMIYNVINRPSGVSNRFSGSKSGNTASLIISGLQAEDEAEYYCSSYIGTNNFGVYVFGTGTKVTV

SEQ ID NO: 91 - protein, 126 aa, synthetic construct
  REGION 1..126: note = heavy chain S.3.2.D9
EVQLVESGGGLVQPGGSQRLSCVVSGFTVSTFYMSWVRQAPGKGLEWVSVIFSGDSTYYADSVKGRFTISRDDSKNILYLQMNSLRAEDTAVYFCARSLKGAYSTSWYFYYAMDVWGQGTTVTVSS

SEQ ID NO: 92 - protein, 108 aa, synthetic construct
  REGION 1..108: note = light chain S.3.2.D9_K
DIVMTQSPATLSLPPGERATLSCRASRSISSNVAWYQQKPGQAPRLLIYDASNRATGIPARFSGSGSGADFTLTISSLEPEDFAFYYCQQRSSLPPLTFGGGTKLEIK

SEQ ID NO: 93 - protein, 118 aa, synthetic construct
  REGION 1..118: note = heavy chain S.8.1.C12
QVQLVQSGAEVKKPGSSVKVSCKASGGTFSSYVIGWVRQAPGQGLEWMGGIIPIFGTTNYAQKSQGRVTITADESSSTAYMELSGLRSEDTAVYYCAGLSQWELMIRWGQGTLVTVSS

SEQ ID NO: 94 - protein, 109 aa, synthetic construct
  REGION 1..109: note = light chain S.8.1.C12_K
EIVLTQSPGTLSLSPGERATLSCRASQSISSSYLAWYQQRPGQAPRLLIYGASSRATGVPDRFSGSGSGTDFTLTISRLEPEDFAVYYCQQYGLSPAWTFGQGTKVEIK

SEQ ID NO: 95 - protein, 117 aa, synthetic construct
  REGION 1..117: note = heavy chain S.8.1.C2
EVQLVESGGGLVQPGGSLRLSCVVSGIIVSNNYMSWVRQAPGKGLEWVAVIYSGGSTFYADSVKGRFTISRHNSKNTLYLQMNSLRTEDTALYYCARDLGNSEFDYWGQGTLVTVSS

SEQ ID NO: 96 - protein, 109 aa, synthetic construct
  REGION 1..109: note = light chain S.8.1.C2_K
DIQLTQSPSSLSASVGDRVTITCRASQGISTYLAWYQQKPGKAPKLLIYAASTLQSGVPSRFSGSGSGTDFTLTISSLQPEDFATYYCQQLNSYPSSYTFGQGTKLEIK

SEQ ID NO: 97 - protein, 116 aa, synthetic construct
  REGION 1..116: note = heavy chain S.9.1.B7
EVQLVESGGGLVQPGGSLRLSCAASGFTVSSNYMSWVRQAPGKGLEWVSVIYSGGSTFYADSVKGRFTISRDNSKNTLYLQMNSLRAEDTAVYYCARDLRGYNDYWGQGTLVTVSS

SEQ ID NO: 98 - protein, 108 aa, synthetic construct
  REGION 1..108: note = light chain S.9.1.B7_K
IQMTQSPSSVPASVGDRVTITCRASQGISSWLAWYQQKPGKAPKLLIYAASSLQSGVPSRFSGSGSGTDFTLTISSLQPEDFATYYCQQTNDFPPALGQGTKVEIKRT

SEQ ID NO: 99 - protein, 117 aa, synthetic construct
  REGION 1..117: note = heavy chain S.9.1.G7
EVQLVETGGGLIQPGGSLRLSCAASGLTVSSNYMSWVRQAPGKGLEWVSVIYAGGSTFYADSVKGRFTISRDNSKNTLYLQMNGLRADDTAVYYCARDLVVYGMDVWGQGTTVTVSS

SEQ ID NO: 100 - protein, 106 aa, synthetic construct
  REGION 1..106: note = light chain S.9.1.G7_K
DIQLTQSPSFLSASVGDRVTITCRASQGISSYLAWYQQKPGKAPKLLIYAASTLQSGVPSRFSGSGSGTEFTLTISSLQPEDFATYYCQHLNSYPAFGQGTKVEIK

SEQ ID NO: 101 - protein, 120 aa, synthetic construct
  REGION 1..120: note = heavy chain S.9.3.A7
QLQLQESGPGLVKPSETLSLTCTVSGGSISSSSYYWGWIRQPPGKGLEWIASLFYSGSTYYNPSLKSRVTISVDTSKNRFFLIPTSVTAADTAVYYCARDSSGSYSIDYWGQGTLVTVSS

SEQ ID NO: 102 - protein, 112 aa, synthetic construct
  REGION 1..112: note = light chain S.9.3.A7_L
QSVLTQPPSVSGAPGQRVTISCSGSSSNIGAGYDVHWYQLLPGTAPKLLIYGNSNRPSGVPDRFSGSKSGTSASLAITGLQAEDEADYYCQSYDTSLSALYVFGTGTKVTVL

SEQ ID NO: 103 - protein, 126 aa, synthetic construct
  REGION 1..126: note = heavy chain S.9.4.A9
QVQLVQSGAEVKKPGASVKVSCKASGYTFISYGISWVRQAPGQELEWMGWISAYNGNTNYAQKLQGRVTMTRDTSTTTAYMELRSLRSDDTAVYYCARVLGGLWFGEPKARHSDYWGQGTLVTVSS

SEQ ID NO: 104 - protein, 106 aa, synthetic construct
  REGION 1..106: note = light chain S.9.4.A9_K
IQMTQSPSSLSASVGDRVTITCRASQGINNYLAWFQQKPGKAPKSLIYAASSLHSGVPSRFSGSGSGTDFTLTISSLQPEDFATYYCQQYNTYPITFGQGTRLEIK

SEQ ID NO: 105 - protein, 128 aa, synthetic construct
  REGION 1..128: note = heavy chain S.9.4.C6
QVQLVQSGSELKKPGASVKVSCKASGYTFTNYAMNWVRQAPGQGLEWMGWIDTNAGNPTYAQGFTGRFVFSLDTSVSTAYLQISSLKPEDTAVYFCARVQGVGVVTKSYYYYYAMDVWGQGTTVTVSS

SEQ ID NO: 106 - protein, 105 aa, synthetic construct
  REGION 1..105: note = light chain S.9.4.C6_L
SYELTQSPSVSVAPGKTARITCGGNDIGSKSVHWYQQRPGQAPVLVVYDDTDRPSGIPERFSGSNSGNTATLTISRVEAGDEADYYCQVWDSSGVFSGGTKLTVL

SEQ ID NO: 107 - protein, 123 aa, synthetic construct
  REGION 1..123: note = heavy chain S.11.1.D4
QVQLVESGGGVVQPGRSLRLSCVASGFSFSTYTMNWVRQAPGKGLEWVTKISSDGTLKDYADSVKGRFTVSRDNYESTLYLEMNSLRTEDTAVYYCARTSGRGSEDRGRFDPWGQGTLVTVSS

SEQ ID NO: 108 - protein, 111 aa, synthetic construct
  REGION 1..111: note = light chain S.11.1.D4_K
DIVMTQSPLSLPVTPGESASISCRSSQSLLHSNGYNYLDWYLQKPGQSPQLLIYLGSNRASGVPDRFSGSGSGRDFTLKISRVEAEDVGVYYCMQSLQTFTFGPGTKVDIK

SEQ ID NO: 109 - protein, 121 aa, synthetic construct
  REGION 1..121: note = heavy chain S.11.1.E10
EVQLVESGGGLVQPGRSLRLSCEVSGFTFEDYAMHWVRQPPGKGLEWVSGISWNGDSIGYAGAVRGRFTISRDNAKNSLSLQMNSLRVEDTALYYCVKGRYVDWTNPLDVWGQGTTVTVSS

SEQ ID NO: 110 - protein, 108 aa, synthetic construct
  REGION 1..108: note = light chain S.11.1.E10_L
SYELTQPPPVSVAPGKTARITCGGDNIGGKSVHWYQQKPGLAPVMVVYDDSARPSGIPERFSGSNSGNTATLTITRAEAGDEADYYCQVWDTGSDPLVFGTGTKVTVL

SEQ ID NO: 111 - protein, 125 aa, synthetic construct
  REGION 1..125: note = heavy chain S.11.1.F1
QLQLQESGPGLVKPSETLSLTCTVSGGSISSSSYYWGWIRQTPGKGLEWIGSIYYSGSTYYRPSLKSRVTISVDTSKNQFSLKLSSVTAADTAVYYCARLARFLEWQPIVSFDYWGQGTLVTVSS

SEQ ID NO: 112 - protein, 110 aa, synthetic construct
  REGION 1..110: note = light chain S.11.1.F1_L
QSALTQPASVSGSPGQSIAISCTGTSSDVGSYNYVSWYQQHPGKAPKLMIYEVSKRPSGVSNRFSGSKSGNTASLTISGLQAEDEADYYCCSYAGSSTVLFGGGTKLTVL

SEQ ID NO: 113 - protein, 117 aa, synthetic construct
  REGION 1..117: note = heavy chain S.11.2.B6
EVQLVESGGGLVQPGGSLRLSCAASEIIVSRNYMNWVRQAPGKGLEWVSVMYPGGSTFYANSVKGRFTISRDNSQNTLFLQMNSLRAEDTAVYYCARDRGNDAFDVWGQGTMVTVSS

SEQ ID NO: 114 - protein, 108 aa, synthetic construct
  REGION 1..108: note = light chain S.11.2.B6_K
DIQLTQSPSFLSASVGDRVTITCRASQGISTYLAWYQQKPGKAPNLLIYAASTLHSGVPSRFSGSGSGTEFTLTISSLQPEDFATYYCQQLNGYPGSNFGQGTKVEIK

SEQ ID NO: 115 - protein, 117 aa, synthetic construct
  REGION 1..117: note = heavy chain S.11.2.E5
EVQLVESGGGLIQPGGSLRLSCAASEIIVSSNYMNWVRQAPGRGLEWVSVIYSGGSTFYADSVKGRFTISRDNSKNTLYLQMNSLRADDTAIYFCARDPYGGAFDVWGQGILVTVSS

SEQ ID NO: 116 - protein, 106 aa, synthetic construct
  REGION 1..106: note = light chain S.11.2.E5_K
DIQMTQSPSTLSASVGDRVTITCRASESFSNWLAWYQQKPGKAPKLLIYQASTLESGVPSRFSGSGSGTEFTLTISSLQPEDFATYYCQQYNSGYTFGQGTKLEIK

SEQ ID NO: 117 - protein, 124 aa, synthetic construct
  REGION 1..124: note = heavy chain S.11.2.F5
QVQLVESGGGVVQPGRSLRLSCAASGFTFSSYVIHWVRQAPGKGLEWVAVISHDGSNKYYADSVKGRFTISRDNSKNTLYLQMNSLRAEDTAVYYCARDRELGKSYGLDAYDIWGQGTMVTVSS

SEQ ID NO: 118 - protein, 103 aa, synthetic construct
  REGION 1..103: note = light chain S.11.2.F5_K
DIQMTQSPSTLSASVGDRVTITCRASQSISSWLAWYQQKPGKAPKLLIYKASSLESGVPSRFSGSGSGTEFTLTISSLQPDDFATYYCQQSQTFGQGTKVEIK

SEQ ID NO: 119 - protein, 121 aa, synthetic construct
  REGION 1..121: note = heavy chain S.11.5.A2
QVQLVQSGAEVKKPGSSVKVSCKASVGTFSSYAISWVRQAPGQGLEWMGRIIPIFGTADYAQKFQGRVTITADESTNTAYMELSSLRSEDTAVYYCARDLETSPLYGMEVWGQGTTVTVSS

SEQ ID NO: 120 - protein, 107 aa, synthetic construct
  REGION 1..107: note = light chain S.11.5.A2_K
DIQMTQSPSSLSASVGDRVTITCRASQSISRFLNWYQQKPGKAPKLLIYATSNLQTGVPSRFSGSGSGTDFTLTISSLQPEDFATYFCQQTYNTPHTFGQGTKLEIK

SEQ ID NO: 121 - protein, 124 aa, synthetic construct
  REGION 1..124: note = heavy chain S.11.5.C7
QVQLQESGPGLVKPSQTLSLTCSVSGDSISINAYYWSWIRQHPGRGLEWIGYMDYSGTTSYSPSLKSRVSISVDTSKNQFSLKLSSVTVADTAVYYCARVGFSYGNPLDAFDVWGQGTMVTVSS

SEQ ID NO: 122 - protein, 112 aa, synthetic construct
  REGION 1..112: note = light chain S.11.5.C7_L
QSVLTQSPSVSGAPGQRVTISCTGSSSNIGAGYDVHWYQQLPGTAPKIIIYANTNRPSGVPDRFSGSKSGTSASLAITGLQAEDEADYYCQSYDSSLSGYVVFGGGTKLTVL

SEQ ID NO: 123 - protein, 117 aa, synthetic construct
  REGION 1..117: note = heavy chain
EVQLVETGGGLIQPGGSLRLSCTASGLIVSSNYMIWVRQAPGKGLEWVSVIYPGGSTFYADSVKGRFTISRDNSKNTLYLQMNSLRAEDTAVYYCARDLVEFGMDVWGQGTTVTVSS

SEQ ID NO: 124 - protein, 107 aa, synthetic construct
  REGION 1..107: note = light chain S.11.6.B5_K
DIQLTQSPSFLSASVGDRVTITCRASQGISNYLAWYQQKPGKAPNLLIYGAFILQSGVPSRFSGSGSGTEFTLTISSLQPEDFATYYCQQLNSESRTFGGGTKVEIK

SEQ ID NO: 125 - protein, 117 aa, synthetic construct
  REGION 1..117: note = heavy chain S.11.6.G11
EVQLVETGGGLIQPGGSLRLSCAASGVTVSSNYMSWVRQAPGKGLEWVSVMYSGGSTFYADSVKGRFTISRDNSKNTLYLQMNSLRAEDTAVYYCARDLVIWGMDVWGQGTTVTVSS

SEQ ID NO: 126 - protein, 107 aa, synthetic construct
  REGION 1..107: note = light chain S.11.6.G11_K
DIQLTQSPSFLSASVGDRVTITCRASQGISSYLAWYQQKPGKAPKLLIYAASTLQSGVPTRFSGSGSGTEFTLTISSLQPEDFATYYCQLLNSYPPTFGGGTKVEIK

SEQ ID NO: 127 - protein, 125 aa, synthetic construct
  REGION 1..125: note = heavy chain S.11.7.A11
QVQLVQSGTEVKKPGSSVKVSCMASGGSFSTSAISWVRQAPGQGLEWMGGIIPITGTASYAQNFQGRVTITADESTSTAYMELSSLRSEDTAVYYCARGYRYCNSTRCYPWFDPWGQGTLVTVSS

SEQ ID NO: 128 - protein, 107 aa, synthetic construct
  REGION 1..107: note = light chain S.11.7.A11_K
DIQMTQSPSSLSASVGDRVTITCRASQSVSSYLNWYQQKSGKAPKLLIYAASSLQSGVPSRFSGSGSGTDFTLTISSLQPEDFATYFCQQSYRSPLTFGGGTKVEIK

SEQ ID NO: 129 - protein, 121 aa, synthetic construct
  REGION 1..121: note = heavy chain S.11.7.A5
EVQLVESGGGLVQPGRSLRLSCAASGFNFDDYAMHWVRQGPGKGLEWVSGISYNSDSIGYAASVKGRVTISRDNAKNSLYLQMNSLRAEDTALYYCAKGRYFDWTHAMDVWGQGTTVTVSS

SEQ ID NO: 130 - protein, 108 aa, synthetic construct
  REGION 1..108: note = light chain S.11.7.A5_L
SYELTQPPSVSVAPGKTARITCGGNNIGSKSVNWYQQRPGQAPVLVVYDDSDRPSGIPERFSGSNSGNTATLTISRVEAGDEADYYCQVWDTGSDPLVFGTGTKVTVL

SEQ ID NO: 131 - protein, 136 aa, synthetic construct
  REGION 1..136: note = heavy chain S.11.7.C8
QVQLVQSGAEVKKPGSSVKVSCKASGGTFSTYAFNWVRQAPGQGLEWMGGIIPMFGTTHDALGFQGTNYAQRFQGRLTITADQSTNTAYMELSGLRSDDTAVYYCARGVPVWGSNGPLGYRAMDVWGQGTTVTVSS

SEQ ID NO: 132 - protein, 107 aa, synthetic construct
  REGION 1..107: note = light chain S.11.7.C8_K
DIQLTQSPSFLSASVGDRVTITCRASQGISSYLAWYQQKPGKAPKLLIYASSTLQSGVPSRFSGSESGTEFTLTISSLQPEDFATYYCQQLNSYPLTFGGGTKVEIK

SEQ ID NO: 133 - protein, 121 aa, synthetic construct
  REGION 1..121: note = heavy chain S.11.7.F5
QVQLVQSGAEVKKPGSSVKVSCKASGGTFSSHAFSWVRQAPGQGLEWMGGIIPIFGTSHYAQKFQGRVTITADESTSTAYMELISLRSDDTAVYYCARYPYDILTGYLDYWGQGTLVTVSS

SEQ ID NO: 134 - protein, 107 aa, synthetic construct
  REGION 1..107: note = light chain S.11.7.F5_L
SYELTQPPSVSVAPGKTARITCGGANIGSKNVHWYQQKPGQAPVLVVYDDSDRPSGIPERFSGSNSGNTATLTISRVEAGDEADYYCQVWDSGNFWVFGGGTKLTVL

SEQ ID NO: 135 - protein, 120 aa, synthetic construct
  REGION 1..120: note = heavy chain S.11.7.G2
  SITE 9: note = misc_feature - Xaa can be any naturally occurring amino acid
QVQLVESGXGVVQPGRSLRLSCAASGFTFSNYAIHWVRQAPAKGLEWVAVILSDGSGKFYADSVKGRFTISRDNSKNTLYLQMNSLRPDDTALYYCARDQGELTTYFDYWGQGTLVTVSS

SEQ ID NO: 136 - protein, 108 aa, synthetic construct
  REGION 1..108: note = light chain S.11.7.G2_K
DIQMTQSPSSLSASVGDRVTITCRASQSIGKYLNWYQQKPGKAPKLLIYVASNLQSGVPSRFSGSGSGTDFTLTISSLQPEDFATYYCQQSYETPPWTFGQGTKVEIK

SEQ ID NO: 137 - protein, 119 aa, synthetic construct
  REGION 1..119: note = heavy chain S.11.7.G3
EVQLVESGGGLFQPGGSLRLSCEVSGFPFSNYWMNWVRQAPGKGLVWISRISSDGSSATYADSVRGRLIISRDNAKNTLYLQMNSLRADDTAVYYCARSEYLRGWFDPWGQGTLVTVSS

SEQ ID NO: 138 - protein, 111 aa, synthetic construct
  REGION 1..111: note = light chain S.11.7.G3_L
NFMLTQPQSVSASPGKTVTISCTGSGGDVINNYVQWYQQRPGSAPTTVIFEDSQRPSGVPDRFSGSIDSSSNSASLTISGLKTEDEADYYCQSFDSRVHVVFGGGTKLIVL

SEQ ID NO: 139 - protein, 123 aa, synthetic construct
  REGION 1..123: note = heavy chain S.11.7.H6
QVQLVQSGAEVKKPGASVKISCEASGYSFTSYYMHWVRQAPGQGLEWMGIIYPSGGRTDYAQKFQGRVTVTRDTSTSTVYLELTSLRSEDTAVYYCARDAKDIVGATLPGCHWGQGTLVTVSS

SEQ ID NO: 140 - protein, 113 aa, synthetic construct
  REGION 1..113: note = light chain S.11.7.H6_K
DIVMTQSPDSLAVSLGERATINCKSSQSLLYISNNKNYLAWYQQKPGQPPKLLIYWASTRESGVPDRFSGSGSGTDFTLTISSLQAEDVAVYYCQHYYSSPITFGQGTRLEIK

SEQ ID NO: 141 - protein, 127 aa, synthetic construct
  REGION 1..127: note = heavy chain S.11.3.D10
EVQLVQSGAEVKKPGESLKISCKASGYIFTNYWIAWVRQMPGKGLEWMGIIYPDDSDTRYGPSFQGQVTISADKSISTAYLQLSSLKASDNAMYYCARHWRPTIAARPGYSYYMDVWGKGTTVTVSS

SEQ ID NO: 142 - protein, 107 aa, synthetic construct
  REGION 1..107: note = light chain S.11.3.D10_K
  SITE 11: note = misc_feature - Xaa can be any naturally occurring amino acid
DIQMTQSPSSXSASVGDRVTITCQASQDIDIYLNWYQQTPGKPPKLLIFDASNLETGVPSRFSGSGSGTDFSFTISRLQPEDTATYYCQQSDSLPLTFGGGTKVEIK

SEQ ID NO: 143 - protein, 123 aa, synthetic construct
  REGION 1..123: note = heavy chain
QVQLVESGGGVVQPGRSLRLSCAASGFGLNTYVMNWVRQSPGKGLQWVAGISSDGSKEQYADSVKGRFTISRDNYENALYLQMNSLRTEDTAVYYCARTSGRGFADRGRFDPWGQGTLVTVSS

SEQ ID NO: 144 - protein, 111 aa, synthetic construct
  REGION 1..111: note = light chain S.11.3.G9_K
DIVMTQSPLSLPVTPGEPASISCRSSQSLLDSNGKNYLDWYLQKPGQSPQLLIYLGSNRASGVPDRFSGSGSGTDFTLKISRVEAEDVGVYYCMEALQTFTFGPGTKVDIK

SEQ ID NO: 145 - protein, 117 aa, synthetic construct
  REGION 1..117: note = heavy chain S.11.3.H8
EVQLVETGGGLIQPGGSLRLSCAVSELIVSVNYMSWVRQAPGKGLEWVSIIYSGGSMFYAGSVKGRFTISRDHSKNTLYLQMNSLRVDDTAVYYCARSYGDFYLDLWGQGTLVTVSS

SEQ ID NO: 146 - protein, 125 aa, synthetic construct
  REGION 1..125: note = light chain S.11.3.H8_K
QLQLQESGPGLLKPSETLSLTCSVSGGSISSSSYYWGWIRQAPGKGLEWIGNIFYSGTAYSSPSLQSRVTMSVDTSKNQFSLNVRSVTAADTAVYYCARLARFLEGQPTASFDYWGPGALVTVSS

SEQ ID NO: 147 - protein, 125 aa, synthetic construct; identical to SEQ ID NO: 146
  REGION 1..125: note = heavy chain S.11.4.A5

SEQ ID NO: 148 - protein, 110 aa, synthetic construct
  REGION 1..110: note = light chain S.11.4.A5_L
QSALTQPASVSGSPGQSITISCTGTSADVGSYNFVSWYQQHPGKAPKLMIYEVSKRPSGVSYRFSGSKSGNTASLTISGLQADDEADYYCYSYVGSTTVLFGGGTKLTVL

SEQ ID NO: 149 - protein, 124 aa, synthetic construct
  REGION 1..124: note = heavy chain S.11.4.A6
QVQLQESGPGLVKPSQTLSLTCSVSGDSISINAYYWNWIRQHPGKGLEWIGYMDYSGSTSYSPSLKSRVSISVDTSKNQFSLKLSSVTVADTAVYYCARVGFSYGNPLDAFDVWGQGTMVTVSS

SEQ ID NO: 150 - protein, 112 aa, synthetic construct; identical to SEQ ID NO: 122
  REGION 1..112: note = light chain S.11.4.A6_L

SEQ ID NO: 151 - protein, 121 aa, synthetic construct
  REGION 1..121: note = heavy chain S.11.4.B5
QVQLQESGPGLVKPSQTLSLTCSVSGGSVTSGGYYWSWTRQYPGRGLEWVGNIYHSGSTNYHPSLRSRTTILVDTSKDQFSLKLSSVTAADTAVYYCARDPVAGRGQFDRWGQGILVTVSS

SEQ ID NO: 152 - protein, 108 aa, synthetic construct
  REGION 1..108: note = light chain S.11.4.B5_K
DIQMTQSPSSLSASVGDRVTITCQASQDISNYLNWYQQKPGKAPKLLIYDASHLETGVPSRFSGSGSGTHFTFTISSLQPEDVATYYCQQCDNLPPPTFGQGTKLEIK

SEQ ID NO: 153 - protein, 117 aa, synthetic construct
  REGION 1..117: note = heavy chain S.11.4.C6
EVQLVESGGGLIQPGGSLRLSCAASEFIVSKNYMSWVRQAPGKGLEWVSVIYPGGTTYYADSVKGRFTISRDSSKNTLYLQMNSLKAEDTALYYCARDFGDFYFDYWGQGTLVTVSS

SEQ ID NO: 154 - protein, 107 aa, synthetic construct
  REGION 1..107: note = light chain S.11.4.C6_K
EIVMTQSPATLSVAPGERATLSCRASQSISSNLAWYQQKPGQAPRLLIYDASTWATDIPARFSGSGSGTEFTLTISSLQSEDSAVYYCQQYYDRPRTFGRGTKVEIK

SEQ ID NO: 155 - protein, 123 aa, synthetic construct
  REGION 1..123: note = heavy chain S.11.4.D7
QVQLVESGGGVVQPGRSLRLSCGASGFPFITYTMNWVRQAPGKGLEWVALISSDGSNKYYADFAKGRFTISRDNYDNTLYLQMNSLRSEDTAVYWCARTGGRGSEDRGRLDAWGQGTLVTVSS

SEQ ID NO: 156 - protein, 111 aa, synthetic construct
  REGION 1..111: note = light chain S.11.4.D7_K
DIVMTQSPLSLPVTPGEPASISCRSSQSLLHTNGHNYLDWYLQKPGQSPQLLIYLGSIRASGVPDRFSGSGSGTDFTLKISRVEAEDVGVYYCMKTLQPFTFGPGTKVDIK

SEQ ID NO: 157 - protein, 132 aa, synthetic construct
  REGION 1..132: note = heavy chain S.11.4.E7
QVQLVQSGAEVKKPGASVTVSCEASGFPFTNYYIHWVRQAPGQGLQWMGLINPSGGSTTYAQKFQGRLTMTRDTSAPIVYMELSSLTSEDTAVYYCARDSPPSVHHCGGDCLSPRYNWFDPWGQGTLVTVSS

SEQ ID NO: 158 - protein, 107 aa, synthetic construct
  REGION 1..107: note = light chain S.11.4.E7_K
EIVLTQSLATLSVSPGERATLSCRASQSVSSNLAWYQQKPGQAPRLLIYGTSIRATGIPARFSGSGSGTEFTLTISSLQSQDFVLYYCQQYNNWPLTFGGGTKVEIK

SEQ ID NO: 159 - protein, 117 aa, synthetic construct
  REGION 1..117: note = heavy chain S.11.4.G9
EVQLVETGGGLIQPGGSLRLSCAASGVTVSSNYMTWVRQAPGKGLEWVAVIYSGGSTFYADSVKGRFTISRDNSKNTLFLQMNSLRAEDTAVYYCARDLVYYGMDVWGQGTTVTVSS

SEQ ID NO: 160 - protein, 107 aa, synthetic construct
  REGION 1..107: note = light chain S.11.4.G9_K
DIQLTQSPSFLSASVGDRVTITCRASQGISNYLAWYQQKPGKAPKLLIYAASTLQSGVPSRFSGSGSGTEFTLTISSLQPEDCATYYCQQLNSHPPAFGQGTKVEIK

SEQ ID NO: 161 - protein, 120 aa, synthetic construct
  REGION 1..120: note = heavy chain S.11.5.D12
QVQLVESGGGVVQPGRSLTISCVASGFSFSTFSMHWVRQTPGKGLEWVAVILYDGSYKSYADSVKGRFTVSRDNSKNTLYLHMNSPKVEDSAVYYCARDFGEMTTHFDYWGQGTLVTVSS

SEQ ID NO: 162 - protein, 108 aa, synthetic construct
  REGION 1..108: note = light chain S.11.5.D12_K
DIQMTQSPSSLSASVGDRVSITCRASHSIGKSLNWYQQIPGKAPKLLIFDTSNLQSGVPSRFSGSGSGTDFTLTINSLQPEDFATYYCQQSYSTPPWTFGQGTKVEIK

SEQ ID NO: 163 - protein, 123 aa, synthetic construct
  REGION 1..123: note = heavy chain S.11.6.B6
QVQLVQSGPEVKKPGSSVKVSCKASGFTFSSSAVQWVRQGRGHRLEWIGWIVVGSGNTNYVQKFQERVTISRDMSTNTAYMELSGLRSEDTAVYYCAAPSCSNVLCFDGFDLWGQGTMVTVSS

SEQ ID NO: 164 - protein, 108 aa, synthetic construct
  REGION 1..108: note = light chain S.11.6.B6_K
EIVLTQSPGTLSLSPGERATLSCRASQSVRSGYFGWYQQKPGQAPRLLIYNASSRATGIPDRFSGSGSGTDFILTISGLGPEDFAVYYCQQYDSSPWAFGQGTKVEIK

SEQ ID NO: 165 - protein, 120 aa, synthetic construct
  REGION 1..120: note = heavy chain S.11.7.B11
EVQLVESGPGLVKPSETLSLTCTVSGVSIRSYYWSWIRQPPGKGLEWIGYIFYSGSTNYNPSLKSRVTISVDTSKNQFSLKLSSVTAADTAVYYCASLGYGDKSWYFELWGRGTLVTVSS

SEQ ID NO: 166 - protein, 108 aa, synthetic construct
  REGION 1..108: note = light chain S.11.7.B11_L
SYELTQPPSVSVAPGMTARITCGGSNIETKSVHWYQKKPDQAPVLVAYDDSDRPSGIPERFSGSNSGNTATLTISRVEAGDEADYYCQVWDSSSDHGVFGGGTKLTVL

SEQ ID NO: 167 - protein, 123 aa, synthetic construct
  REGION 1..123: note = heavy chain S.11.7.D12
QVQLVESGGGMVQPGRSLRLSCAASGFPFITYTMHWIRQAPGKGLEWVAGVSSDGSDVYSADSVKGRLTISRDNFVNTLHLQMNSLKTDDTAVYYCARTGGRGSQDRGRFDLWGQGTLVTVSS

SEQ ID NO: 168 - protein, 111 aa, synthetic construct
  REGION 1..111: note = light chain S.11.7.D12_K
DIVMTQSPLSLPVTPGEPASISCRSSQSLLHTNGHNYLDWYLQKPGQSPQLLIYLGSNRASGVPDRFSGSGSGTDFTLKISRVEAEDVGVYYCMQSLQSYTFGPGTKVDIK

SEQ ID NO: 169 - protein, 126 aa, synthetic construct
  REGION 1..126: note = heavy chain S.11.7.E6
QVQLVQSGAEVKKPGSSVKVSCKASGGPFSIYSITWVRQAPGQGLEWMGGIIPMRNTPNYAQKFQGRVTITADASTTTGYMELSSLRSEDTAVYYCARDYRYCNDTTCYGFAFDIWGQGTMVTVSS

SEQ ID NO: 170 - protein, 106 aa, synthetic construct
  REGION 1..106: note = light chain S.11.7.E6_K
DIQMTQSPSSLSASVGDRVTITCRASQSINNFLNWYQQKPGKAPKLLIYAASSLQSGVPSRFGGSGSGTDFTLTISSLQPDDFATYYCQQSYSSRTFGQGTKLEIK

SEQ ID NO: 171 - protein, 124 aa, synthetic construct
  REGION 1..124: note = heavy chain S.11.8.D10
  SITE 123: note = misc_feature - Xaa can be any naturally occurring amino acid
QVQLVESGGGVVQPGRSLRLSCAASGFTFSTYVMHWVRQAPGGGLEWVAVISSDGSNRYNADSVKGRFTISRDNSKNTLYLQMNSLRTEDTAVYFCARDREVGKSYGLDGFDVWGQGTMVTVXS

SEQ ID NO: 172 - protein, 103 aa, synthetic construct
  REGION 1..103: note = light chain S.11.8.D10_K
DIQMTQSPSTLSASVGDRVTITCRASQNISPWLAWYQQKPGRAPKLLIYKASTLESGVPSRFSGSGSGTEFTLTISSLQPDDFATYYCQQLQTFGQGTKVEIK

SEQ ID NO: 173 - protein, 123 aa, synthetic construct
  REGION 1..123: note = heavy chain S.11.8.E10
QVQLVQSGPEVKKPGTSVKVSCKASGFTFSMSAVQWVRQARGQRLEWIGWIVVGSGNTELAQKFQQRVIMTRDESTGTAYMELNSLTSEDTAAYYCAAPSCTNVLCFDGFDLWGQGTMVTVSS

SEQ ID NO: 174 - protein, 108 aa, synthetic construct
  REGION 1..108: note = light chain S.11.8.E10_K
EIVLTQSPGTLSLSPGERATLSCRASQSVRSSYLGWYQQKPGQAPRLLMYNTSSRATGIPDRFSGSGSGTAFTLTITRLEPEDIGVYHCQQYDRSPWTFGQGTKVEIK

SEQ ID NO: 175 - protein, 118 aa, synthetic construct
  REGION 1..118: note = heavy chain S.11.8.H11
EVQLVETGGGLIQPGGSLRLSCTTSGLIVSRNYMHWVRQAPGKGLEWVAVIYPGGTTHYADSVKGRFTISREHSNNTLSLQMKSLRAGDTAVYYCARDLDVLGGFDIWGQGTMVTVSS

SEQ ID NO: 176 - protein, 107 aa, synthetic construct
  REGION 1..107: note = light chain S.11.8.H11_K
AIRMTQSPSSFSASTGDRVTISCRTSQDINNDLAWYQQKPGKAPNLLIYGASTLQTGVPSRFSGSGSGTEFTLTITYVKSEDFATYYCQQYSNYPRTFGQGTKVEIK

SEQ ID NO: 177 - protein, 119 aa, synthetic construct
  REGION 1..119: note = heavy chain S.11.8.D6
QVQLVESGGGVVQPGRSLRLSCAASGFTFSIYGMHWVRQAPGKGLEWVAVMSYDGSHVYYGDSVKGRFTISRDNSKNTLYLQMNILRVEDTAVYYCARDYGDYAALDHWGQGTLVTVSS

SEQ ID NO: 178 - protein, 112 aa, synthetic construct
  REGION 1..112: note = light chain S.11.8.D6_K
DIVMTQSPDSLAASLGERATINCKSSQSVLYNSNNKNYLAWYQQKPGQPPKLLIYWASIRESGVPDRFSGSGSGTDFTLTISSLQAEDVAFYYCQPYLPTPTFGPGTKVDIK

SEQ ID NO: 179 - protein, 124 aa, synthetic construct
  REGION 1..124: note = heavy chain S.11.4.A8
QVQLQESGPGLVKPSETLSLTCAVSGYSISSGYYWGWIRQPPGKGLEWIGSMHHSGNTDYNPSLKSRATISIDTSKNQLSLKLSSVTAADTAVYYCARIMQGRIVVLISYIDFWDQGSLVTVSS

SEQ ID NO: 180 - protein, 111 aa, synthetic construct
  REGION 1..111: note = light chain S.11.4.A8_L
QSVLTQPPSASGTPGQRVTISCSGGSSNIGRNTVDWYQQLPGTAPKLLIYSSNQRPSGVPDRFSGSKSGTSASLAISGLQSGDEADYYCASWDDTLNGQLVFGGGTKLTVL

SEQ ID NO: 181 - protein, 122 aa, synthetic construct
  REGION 1..122: note = heavy chain S.8.2.B2
EVQLVESGGGWVQPGGSLRLSCSASGFSFSTYAMNWVRQAPGKGLEYVSGISSNGDITYYADSVKGRFTISRDNSKNTLYLQMSSLRTEDTAIYYCVKDLGTVVTVDVFDIWGQGTMVTVSS

SEQ ID NO: 182 - protein, 107 aa, synthetic construct
  REGION 1..107: note = light chain S.8.2.B2_K
DIQMTQSPSSLSASVGDRVTITCRPSQTINSYLNWYQQKPGKAPKLLIYAASSLQSGVPSRFSGSGSGTDFTLTISSLQPEDFATYYCQQTYITPGTFGQGTKVEIK

SEQ ID NO: 183 - protein, 123 aa, synthetic construct
  REGION 1..123: note = heavy chain S.9.1.C11
QVQLVQSGAEVKKPGASVRVSCKTSGYTFTTYFIHWVRQAPGRGLEWMGIINPSGGSTSYALKFQGRVTMTRDTSTSTVYMELSSLRSEDTAVYYCAREEDIVVVPAASFDYWGQGTLVTVSS

SEQ ID NO: 184 - protein, 109 aa, synthetic construct
  REGION 1..109: note = light chain S.9.1.C11_K
EIVLTQSPATLSLSPGERATLSCRASQSVSSYFAWYQQKPGQSPRLLIYDASNRASGIPARFSGSGSGTDFTLTISSLEPEDFAVYYCQQRSNWPPRITFGQGTRLEIK

SEQ ID NO: 185 - protein, 129 aa, synthetic construct
  REGION 1..129: note = heavy chain S.9.1.D10
QVQLQESGPGLVKPSETLSLTCSVSGGSINNYYWSWIRQPPGKGLEWIGYIYFSGNTNYNPSLKSRVTISIDTSKNQFSLKLSSVTAADTAVYYCAREGTGYCSGGTCYSAEEDAFDIWGQGTMVTVSS

SEQ ID NO: 186 - protein, 107 aa, synthetic construct
  REGION 1..107: note = light chain S.9.1.D10_K
DIQMTQSPSSLSASVGDRVTITCRASQSISRYLNWYQQKPGKAPKLLIYTASSLQSGVPSRFSGSGSGTDFTLTISSLQPEDFATYYCQQSHSTPWTFGQGTKVEIK

SEQ ID NO: 187 - protein, 124 aa, synthetic construct
  REGION 1..124: note = heavy chain S.9.2.B2
QVQLQESGPGLVKPSQTLSLTCTVSGGSISSGDYYWSWIRQPPGKGLEWIGYIYYSGSTYYNPSLRSRVSISVDTSKNQLSLKLRSVTAADTAVYYCARDHGGGYNWGPGFDSWGQGTLVTVSS

SEQ ID NO: 188 - protein, 107 aa, synthetic construct
  REGION 1..107: note = light chain S.9.2.B2_K
DIQMTQSPSSLSAYVGDRVTITCRASQNISSYLNWYQQKPGKAPKFLIYAASSLQSGVPSRFSGSGSGTNFTLTVSSLQPEDFATYYCQQSYSTLWTFGQGTKVEIK

SEQ ID NO: 189 - protein, 130 aa, synthetic construct
  REGION 1..130: note = heavy chain S.9.3.H9
EVQLVESGGGLVKPGGSLRLSCAASGFSFSSYSMNWVRQTPGKGLEWVSSISSSSTSFIYYADSVMGRFTISRDNAKNSLYLQMNRPRAEDTAVYYCARDFTPSPRRYFDWLLPLGMDVWGQGTTVTVSS

SEQ ID NO: 190 - protein, 110 aa, synthetic construct
  REGION 1..110: note = light chain S.9.3.H9_L
QSALTQSRSVSGSPGESVAISCTGTSSDVGAYNYVSWYQQHPGKAPKLMIYDVNKRPSGVPDRFSGSKSGNTASLTISGLQAEDEADYYCCSYAGSYNWVFGGGTKLTVL

SEQ ID NO: 191 - protein, 118 aa, synthetic construct
  REGION 1..118: note = heavy chain S.11.1.E2
  SITE 31: note = misc_feature - Xaa can be any naturally occurring amino acid
EVQLVESGGDLVQPGGSLRLSCAASGFSLSXHWMSWVRQVPGKGLEWVANIKHDESETYYVASVKGRFTISRDNAKNSLYLQMNSLTDEDSAIYYCTREAKSGPGDYWGRGTLVTVSS

SEQ ID NO: 192 - protein, 110 aa, synthetic construct
  REGION 1..110: note = light chain S.11.1.E2_L
QSVLTQPPSASGTPGQRVTISCSGSNSNIGSRFVYWYQQLPGTAPTLLIYRDDQRPSGVPDRFSGSKSGTSASLAISGVRSEDEADYYCAVWDDNLTGWVFGGGTKLTVL

SEQ ID NO: 193 - protein, 123 aa, synthetic construct
  REGION 1..123: note = heavy chain S.11.2.C6
QVQLVESGGGVVQPGRSLRLSCAASGFGFNFYLIHWVRQAPGKGLEWVALISFDGTNEYYADSVKGRFIISRDNSENTLYLQMNSLRTEDTAVYYCARTGGRGSADRGRFDLWGQGTLVTVSS

SEQ ID NO: 194 - protein, 110 aa, synthetic construct
  REGION 1..110: note = light chain S.11.2.C6_K
IVMTQSPLSLSVTPGEPASISCRSSQSLLHSNGHTYLDWYLQKPGQSPQLLIYLGSNRASGVPDRFSGSGSGTDFTLKISRVEAEDVGIYYCMQAIQSFTFGPGTKVDIK

SEQ ID NO: 195 - protein, 124 aa, synthetic construct
  REGION 1..124: note = heavy chain S.11.2.F11
EVQLLESGGGLVQPGGSQRLSCAASGFTFSSYPMSWVRQAPGKGLEWVSFISGSGGTIYYADSVKGRFTISRDNSKNTLYLQMNSLRAEDTAVYYCAKDPSTAPIYYYFYMDVWGKGTTVTVSS

SEQ ID NO: 196 - protein, 112 aa, synthetic construct
  REGION 1..112: note = light chain S.11.2.F11_L
QSALTQPASVSGSPGQSITISCTGTSSNVGGYNLVSWYQKHLGKAPKLMIFDVNKRPSGVSNRFSGSKSGNTASLTISGLQAEDEADYYCCSYAGRSTSYVVFGGGTKLTVL

SEQ ID NO: 197 - protein, 123 aa, synthetic construct
  REGION 1..123: note = heavy chain S.11.3.B3
  SITE 9: note = misc_feature - Xaa can be any naturally occurring amino acid
QVQLVESGXGVVQPGGSRRLSCAASGFGLNTYVLHWVRQPPGKGLEWVALISSDGGNEQFADSVKGRFTISRDNFDNKVFLQMNGLTTEDTAVYFCARTGGRGSADRGRFDLWGHGALVTVSS

SEQ ID NO: 198 - protein, 111 aa, synthetic construct
  REGION 1..111: note = light chain S.11.3.B3_K
DIVMTQSPLFLPVTPGEPASISCRSSQSLLHSNGYNYLDWYLQKPGQSPQLLIYLGSNRASGVPDRFSGSGSGTDFTLKISRVEAEDVGVYYCMEALQAFTFGPGTKVDIK

SEQ ID NO: 199 - protein, 117 aa, synthetic construct
  REGION 1..117: note = heavy chain S.11.3.G8
EVQLVESGGGLIQPGGSLRLSCAASEVIVSSNYMSWVRQAPGKGLEWVSVLFAGGSTFYAASVKGRFTISRDDVKNTLYLQMNSLSAEDTAVYYCARDRWEGAFDIWGLGTMVTVSS

SEQ ID NO: 200 - protein, 108 aa, synthetic construct
  REGION 1..108: note = light chain S.11.3.G8_K
DIQMTQSPSFLSASVGDRVTITCRASQGISNYLAWYQQKPGKAPKLLIYAASTLQSGVPSRFSGSGSGTEFTLTVSSLQPEDFATYYCQQLNSYPKITFGPGTKVDIK

SEQ ID NO: 201 - protein, 124 aa, synthetic construct
  REGION 1..124: note = heavy chain S.11.5.D7
EVQLLESGGGLIQPGGSPRLSCAASGFTFSSSVMTWVRQAPGKGLEWVSAVSGTGGSIYYADSVKGRFTISRDNSKETLYLQMNSLRAEDTAVYYCAKEPPAARYFHHFYMDVWGKGTTVTVSS

SEQ ID NO: 202 - protein, 112 aa, synthetic construct
  REGION 1..112: note = light chain S.11.5.D7_L
QSALTQPASVSGSPGQSITISCTGTSSDVGSYDLVSWYQQHPGKAPELMIYEVTKRPSGVSDRFSGSKSGNTASLTISGLQAEDEADYYCCSYAGRSTSYVVFGGGTKVTVV

SEQ ID NO: 203 - protein, 120 aa, synthetic construct
  REGION 1..120: note = heavy chain S.11.6.F1
QVQLQESGPGLVKASETLSLTCTVSGVSIRSYYWSWIRQPPGKGLEWIGYIFYSGSTNYNPSLKSRVTMSVDTSKNQFSLKLSSVTAADTAVYYCASLGYGDASWYFDLWGRGTLVTVSS

SEQ ID NO: 204 - protein, 108 aa, synthetic construct
  REGION 1..108: note = light chain S.11.6.F1_L
SYELTQPPSVSVAPGKTARITCGGNNIGSKSVHWYLQKPGQAPVLVVYDDSDRPSGIPERFSGSNSGNTATLTISRVEAGDEADYYCQVWDTSSDHGVFGGGTKLTVL

SEQ ID NO: 205 - protein, 122 aa, synthetic construct
  REGION 1..122: note = heavy chain S.11.6.B11
QVQLQESGPGLVTPSGTLSLTCVVSGGSVSSTNWWSWVRQPPGKGLEWIGEIFQSGNTHYNPSLKSRVSMSLDKSNNHFSLTLTSVTAADTAVYYCARGPLLGGGNYYLDVWGKGTTVTVSS

SEQ ID NO: 206 - protein, 111 aa, synthetic construct
  REGION 1..111: note = light chain S.11.6.B11_L
QSALTQPASVSGSPGQSITISCTGTSSDVGSYNLVSWYRQYPGKAPSLMIYQVTKRPSGVSDRFSGSKSGNTASLTIAGLQVEDEGDYYCCSYAGSDTQLLFGGGTKLTVL

SEQ ID NO: 207 - protein, 120 aa, synthetic construct
  REGION 1..120: note = heavy chain S.11.7.B3
QVQLVQSGAEVKKPGASVKVSCKASGYTFTNYHLHWVRQAPGQGPEWMGIFYPSGGSTGYARTFQGRVTMTRDTSTSTVYMELSSLRSDDTAVYYCAREGGSGETYFDYWGQGTLVTVSS

SEQ ID NO: 208 - protein, 109 aa, synthetic construct
  REGION 1..109: note = light chain S.11.7.B3_L
SYELTQPPSVSVAPGKPARITCGGSYIGSKSVHWYQQQPGQAPVLVVYDDSDRPSGIPERFSGSNSGNTATLTISRVEAGDEADYYCQVWDGSSDRQVVFGGGTKLTVL

SEQ ID NO: 209 - protein, 124 aa, synthetic construct
  REGION 1..124: note = heavy chain S.11.7.E9
EVQLLESGGGLVQPGGSLRLSCAASGFTFSSYVVSWVRQAPGKGLEWVSTISGIGISTYYADSVRGRFTISRDKSKNTLYLEMNSLSAEDTAVYYCAKDPSAAAHYYYYYMDVWGKGTTVTVSS

SEQ ID NO: 210 - protein, 112 aa, synthetic construct
  REGION 1..112: note = light chain S.11.7.E9_L
QSALTQPASVSGSPGQSITISCTGTSSDVGNYNLVSWYQQHPGKAPKLMIYEVSKRPSGVSNRFSGSKSGNTASLTISGLQAEDEADYYCCSYAGSSTSYVLFGGGTKLTVL

SEQ ID NO: 211 - protein, 120 aa, synthetic construct
  REGION 1..120: note = heavy chain S.11.7.C11
QVQLVESGGGVVQPGRSLRLSCAASGFIFSNYGMHWVRQAPGKGLEWMAVILDDGSGKFYADSVKGRFTISRDNSKNTLYLQLNSLREDDTAVYYCARDWGSLVTLFDYWGQGTLVTVSS

SEQ ID NO: 212 - protein, 108 aa, synthetic construct
  REGION 1..108: note = light chain S.11.7.C11_K
DIQMTQSPSSLSASVGDRVTITCRASQRIQTYLNWYQQKPGKAPKLLIHSASSLQSGVPSRFSGSGSGTDFTLTISSLQPEDFGTYYCQQSYETPPWTFGQGTKVEIK

SEQ ID NO: 213 - protein, 117 aa, synthetic construct
  REGION 1..117: note = heavy chain S.11.8.F10
EVQLVETGGGLIQPGGSLRLSCAASGVTVSRNYMYWVRQAPGKGLEWVSVIYSGGSTFYADSVKGRFTISRDNSNNTLYLQMNSLRAEDTAVYYCARDAVVYGMDVWGQGTTVTVSS

SEQ ID NO: 214 - protein, 108 aa, synthetic construct
  REGION 1..108: note = light chain S.11.8.F10_K
DIQMTQSPSSLSASVGDRVTITCRASQSISTYLNWYQQKPGKAPKLLIYAASSLQSGVPSRFSGSGSGTDFTLTISSLQPEDFATYYCQQSYSTPPFTFGPGTKVDIK

SEQ ID NO: 215 - protein, 128 aa, synthetic construct
  REGION 1..128: note = heavy chain S.12.1.A4
QVQLVQSGTEVKKPGSSVKVSCKASGGTFSSSAISWVRQAPGQGLEWMGGIITIFGTSNIAQKFQGRVTITADAPSSTAYMGLSSLRSEDTAVYYCARSRGRYYSSSRVYHYYGMDVWGQGTTVTVSS

SEQ ID NO: 216 - protein, 107 aa, synthetic construct
  REGION 1..107: note = light chain S.12.1.A4_K
DIQMTQSPSSLSASVGDRVTITCQARQDISNYLNWYQQKPGKAPKLLIYDASNLETGVPSRFSGRGSGTHFTFTISSLQPEDIATYYCQQYDNLPLTFGGGTKVEIK

SEQ ID NO: 217 - protein, 127 aa, synthetic construct
  REGION 1..127: note = heavy chain S.12.1.B7
QVQLVQSGAEVKKPGSSVKVACRASGDTLSSYAISWVRQAPGQGLEWMGGIIPMFGIADYAHKFQGRVTITADGSTSTAYMELSSLRSEDTAVYYCARTLAGQLGRVNYYYGMDVWGLRGPRSPSPQ

SEQ ID NO: 218 - protein, 112 aa, synthetic construct
  REGION 1..112: note = light chain S.12.1.B7_K
DIVMTQSPLSLPVTPGEPASISCRSSQSLLHSNGYNYLDWYLQKPGQSPQLLIYLGSNRASGVPDRFSGSGSGTDFTLKISRVEAEDVGVYYCMQALQTPPTFGQGTKVEIK

SEQ ID NO: 219 - protein, 117 aa, synthetic construct
  REGION 1..117: note = heavy chain S.12.1.C10
EVQLLESGGDLIQPGGSLRLSCAASGFTFSTYAMIWARQAPGKGLEWVSSITGSGDYTYFADSVKGRFTMSRDNSKNTVYLQMNNLRVEDTALYFCAKGGMTTAYYWGQGTLVTVSS

SEQ ID NO: 220 - protein, 114 aa, synthetic construct
  REGION 1..114: note = light chain S.12.1.C10_K
DIVMTQSPDSLAVSLGERATINCKSSQTILHNSHNRNCLAWFQQKPGQPPKLLIYWASTRESGVPDRFSGSGSGTDFTLTINNLQAEDVAVYYCQQYYTNPRWTFGQGTKVEIK

SEQ ID NO: 221 - protein, 130 aa, synthetic construct
  REGION 1..130: note = heavy chain S.12.2.A3
EVQLVESGGGLVEPGGSLRLSCAASGFTFTSYTMNWVRQAPGKGLEWVSSISSSGRHIHYGDSMKGRFHISRDNSKSLVFLEMNSLRAGDTAMYYCARGYDVLTGYYKIQKSRYYHMDVWGQGTTVTVSS

SEQ ID NO: 222 - protein, 110 aa, synthetic construct
  REGION 1..110: note = light chain S.12.2.A3_L
QSVLTQPPSASGTPGQRVTVSCSGSSSNIGSNTVNWYQQIPGTAPKLLMYGNNQGASGVPDRFSGAKSGTSASLAISGLQSEDEADYYCEAWDDSLNGRVFGTGTKVTVL

SEQ ID NO: 223 - protein, 122 aa, synthetic construct
  REGION 1..122: note = heavy chain S.12.2.C5
QVQLVQSGAEVKKPGASVKVSCKASGYTFTNYYIHWVRQAPGQGLEWMGMINPAGGSIAYAQKFQGRVTMTRDTSTSTVYMDLSSLTSEDTAVYYCARDDFVVPAAGPFDPWGQGTLVTVSS

SEQ ID NO: 224 - protein, 107 aa, synthetic construct
  REGION 1..107: note = light chain S.12.2.C5_K
DIQMTQSPSTLSASVGDRVTITCRASQSISSWLAWYQQKPGKAPKLLIYKASSLQSGVPSRFSGSGSGTEFTLTISSLQPDDFATYYCQHYNGYSKTFGQGTKVEIK

SEQ ID NO: 225 - protein, 126 aa, synthetic construct
  REGION 1..126: note = heavy chain S.12.2.G11
EVQLVESGGGLVKPGGSLRLSCAASGFTFNNAWMNWVRQAPGKGLEWVGRIKSKTDGGTTDYAAPVKGRFTISRDDSENTLFLQMNSLKTEDTAVYYCTTDDSVLWFGELPYFDYWGQGTLVTVSS

SEQ ID NO: 226 - protein, 109 aa, synthetic construct
  REGION 1..109: note = light chain S.12.2.G11_K
EIVLTQSPGTLSLSPGERATLSCRASQSVSSSFLVWYQQKPGQAPRLLMYGASTRATGIPDRFSGSGSGTDFTLTISRLEPEDFAVYYCQHYGNSPPRTFGQGTKVEIK

SEQ ID NO: 227 - protein, 126 aa, synthetic construct
  REGION 1..126: note = heavy chain S.12.3.H1
EVQLVESGGGLVKPGGSLRLSCAVSGFTFSNAWMSWVRQAPGKGLEWVGRVKSKSDGGTTDYAAPVKGRFTISRDDSKNTLYLQMNSLKTEDTAVYYCTTDDSVLWFGELSYFDYWGQGTLVTVSS

SEQ ID NO: 228 - protein, 109 aa, synthetic construct
  REGION 1..109: note = light chain S.12.3.H1_K
EIVLTQSPGTLSLPPGERATLSCRASQSVSSSFLAWYQQKPGQAPRLIMYGASTRATGIPDRFSGSGSGTDFTLTISRLEPEDFAVYYCRHYGNSPPRTFGQGTKVEIK

SEQ ID NO: 229 - protein, 123 aa, synthetic construct
  REGION 1..123: note = heavy chain S.12.1.B12
EVQLVESGGGLVQPGRSLRLSCAASGFTFDDYAMHWVRQAPGKGLEWVSGISWNSGSIGYADSVRGRFTISRDNAKNSLYLQMNSLRTEDTALYYCAKDTHQLVEGDNWFDPWGQGTLVTVSS

SEQ ID NO: 230 - protein, 106 aa, synthetic construct
  REGION 1..106: note = light chain S.12.1.B12_K
IQMTQSPSSVSASVGDRVTITCRASQDISSWLAWYQQKPGRAPKLLIYAASSLQSGVPSRFSGSGSGTDFTLTISSLQPEDFATYYCQQANNFPLTFGGGTKVEIK

SEQ ID NO: 231 - protein, 126 aa, synthetic construct
  REGION 1..126: note = heavy chain S.12.4.A8
EVQLVESGGGLVKPGGSLRLSCAASGFTFTNAWMSWVRQPPGRGLEWVGRIRSKSDGGTTDYAAPVKGRFSISRDDSKNTLYLQMNSLKTEDTAVYYCTTDDSVLWFGELPYFDYWGQGALVTVSS

SEQ ID NO: 232 - protein, 109 aa, synthetic construct
  REGION 1..109: note = light chain S.12.4.A8_K
EIVLTQSPGTLSLSPGERATLSCRASQSISASYLAWYQQKPGQAPRLLMYGASSRATGIPDRFSGSGSGTDFTLTISRLEPEDFAVYYCQQYGSSPPRTFGQGTKVEIK

SEQ ID NO: 233 - protein, 121 aa, synthetic construct
  REGION 1..121: note = heavy chain S.11.1.F6
QVQLQESGPGLVKPSETLSLTCSVSGGSIINSAIWWNWVRQTPGKGLEWIGEVYHRGSTNYNPSLKSRVTLSLDKSKNQFSLKLTSLTAADTAVYYCASKLFDNYIRFESWGQGTLVTVSS

SEQ ID NO: 234 - protein, 108 aa, synthetic construct
  REGION 1..108: note = light chain S.11.1.F6_K
EIVLTQSPGTLALSPGESGTLSCRANESLNSNYVAWLQQKPGQAPRLLIYATSTRATGIPVRFSGSGSGTDFTLTVSSLEPEDFAVYYCQQYDRPPVTFGAGTKVEIK

SEQ ID NO: 235 - protein, 129 aa, synthetic construct
  REGION 1..129: note = heavy chain S.11.3.E5
QLQLQESGSGLVKPSQTLSLTCTVSGGSIGSGGYTWNWIRQAPGKGLESIGYIYPGGSAYYNPSLKSRVTISVDGSKNQFSLKLSSVTAADTAVYYCAREYGIGRGYDDMPVYRRFDLWGRGALVTVSS

SEQ ID NO: 236 - protein, 107 aa, synthetic construct
  REGION 1..107: note = light chain S.11.3.E5_K
DIQMTQSPSSLSASVGDRVSITCRASQNISSYLNWYQQKPGKAPELLIYGAFSLESGVPSRFSGSGSGTDFTLTITSLQPEDFATYSCQQTYGTPRTFGQGTKVEIK

SEQ ID NO: 237 - protein, 123 aa, synthetic construct; identical to SEQ ID NO: 229
  REGION 1..123: note = heavy chain S.12.2.G6

SEQ ID NO: 238 - protein, 106 aa, synthetic construct; identical to SEQ ID NO: 230
  REGION 1..106: note = light chain S.12.2.G6_K

SEQ ID NO: 239 - protein, 122 aa, synthetic construct
  REGION 1..122: note = heavy chain S.11.4.E4
QLQLQESGPGLVKPSETLSLTCTVSGGSLYSGGHFWGWFRQPPGKGLEWIGSVFYSGITYYNPSLEGRLTIFVDPAKNQFSLRLNSVTAADTAVYFCASLYDNSGLWQFDYWGQGTLVTVSS

SEQ ID NO: 240 - protein, 106 aa, synthetic construct
  REGION 1..106: note = light chain S.11.4.E4_K
IQMTQSPSSLSASVGDRVTISCRASQGVGDDLAWYQQKPGRAPKRLIYSASSLQSGVPSRFSGSGYGTEFTLTITSLQPEDFATYYCLQYNSYPLTFGGGTKVEIK

SEQ ID NO: 241 - protein, 117 aa, synthetic construct
  REGION 1..117: note = heavy chain S.11.5.C2
  SITE 75: note = misc_feature - Xaa can be any naturally occurring amino acid
  SITE 77: note = misc_feature - Xaa can be any naturally occurring amino acid
EVQLVESGGGLIQPGGSLRLSCEASGIIVSSNYMTWVRQAPGKGLEWVSVLYAGGSTFYTDSVKGRFTISRDNSXNXLYLQMNSLRAEDTAVYYCARDLAVFGVDIWGQGTMVTVSS

SEQ ID NO: 242 - protein, 109 aa, synthetic construct
  REGION 1..109: note = light chain S.11.5.C2_K
DIQLTQSPSFLSAFVGDRVTITCRASQGISSDLAWYQQQPGKAPKLLIYAASTLQSGVPSRFSGSGSGTEFTLTISSLQPEDFATYYCQHLNSNPGIFTFGPGTKVDIK

SEQ ID NO: 243 - protein, 122 aa, synthetic construct
  REGION 1..122: note = heavy chain S.11.8.G10
  SITE 15: note = misc_feature - Xaa can be any naturally occurring amino acid
  SITE 24: note = misc_feature - Xaa can be any naturally occurring amino acid
QVQLQESGPGLVTPXGTLSLTCVXSGGSVSSTNWWSWVRQPPGKGLEWIGEIFQSGNTHYNPSLKSRLSMSLDKSNNHFSLTLTSVTAADTAVYYCARGPLLGGGNYYLDVWGKGTTVSVSS

SEQ ID NO: 244 - protein, 111 aa, synthetic construct
  REGION 1..111: note = light chain S.11.8.G10_L
QSALTQPASVSGSPGQSITISCTGTSSDIGSYNLVSWYRQYPGEAPSLVIYQVSKRPSGVSDRFSGSKSGNTASLTIAGLQAEDEADYYCCSYAGSDTQLFFGGGTRLTVL

SEQ ID NO: 245 - protein, 124 aa, synthetic construct
  REGION 1..124: note = heavy chain S.12.1.A5
QVQLQESGPRLVRPSQTLSLNCTVSGDSLSRNIIYWTWIRQRPGKGLEWIGYIQHTGTTFYSPSLKSRLIMSIDTSNNQFSLSLDSLTAADTAVYYCVRGIYCGGGCYRGADHWGPGIQVAVSS

SEQ ID NO: 246 - protein, 112 aa, synthetic construct
  REGION 1..112: note = light chain S.12.1.A5_K
DIVMTQSPLSLPVTPGEPASISCRSSQSLLHSNGYTYLDWYLQKPGQSPQLLIYLGSYRASGVPDRFSGSGSGTDFTLKIGRVEAEDVGIYYCMQGLQTPYSFGQGTKLEIK

SEQ ID NO: 247 - protein, 124 aa, synthetic construct
  REGION 1..124: note = heavy chain S.12.1.E10
QVQLQESGPRLVRPSQTLSLNCTVSGDSISRHIIYWTWIRQRPGKGLEWIGYIHHTGSTFYSPSLKSRLTMSIDTSNNQFSLSLGSLTAADTALYYCARGTYCGGACYRGTDHWGPGIQVAVSS

SEQ ID NO: 248 - protein, 112 aa, synthetic construct
  REGION 1..112: note = light chain S.12.1.E10_K
DIVMTQSPLSLPVTPGEPASISCRSSQSLLHNNGYTYLDWYLQKPGQSPQLLIYLGSYRASGVPDRFSGSGSGTDFTLKIGRVEAEDVGIYYCMQGLQTPYSFGQGTKLEIK

SEQ ID NO: 249 - protein, 123 aa, synthetic construct
  REGION 1..123: note = heavy chain S.12.3.E12
QVQLVESGGGLVKPGGSLRLSCAASGFTFSGHYMAWIRQAPGKGLEWLSYISTSGSYTEYVDSVKGRFTISRDNARNSLYLQMNSLRVDDTAIYYCARDHCGADCYSNWFDSWGQGTLVTVSS

SEQ ID NO: 250 - protein, 113 aa, synthetic construct
  REGION 1..113: note = light chain S.12.3.E12_K
DIVMTQSPDSLAVSLGERAAITCKSSQSVLYSSSNRNYLAWYQQKPGQSPKLLIYWASTRASGVPDRFSGSGSETDFTLTISSLQTEDVAVYYCQQYYNTPLTFGGGTKVEIK

SEQ ID NO: 251 - protein, 118 aa, synthetic construct
  REGION 1..118: note = heavy chain S.11.1.B8
EVQLVESGGVLVQPGGSLRLSCAASGFSLSNHWMSWVRQAPGKGLEWVANIKHDGSEKYYVDSVKGRFTISRDNARNSLYLQMDSLRAEDTALYYCAREAFSGPGDYWGQGTLVTVSS

SEQ ID NO: 252 - protein, 110 aa, synthetic construct
  REGION 1..110: note = light chain S.11.1.B8_L
QSVLTQPPSASGTPGQRVTVSCSGRGSNIGNNFVYWYQQLPGTAPKLLIYRNDQRPSGAPDRFSGSKSGTSASLAISGLRSEDEADYYCAAWDDSLRGWVFGGGTKLTVL

SEQ ID NO: 253 - protein, 132 aa, synthetic construct
  REGION 1..132: note = heavy chain S.11.1.E9
  SITE 37: note = misc_feature - Xaa can be any naturally occurring amino acid
EVQLLESGGGLVQPGGSLRLSCAASGFTFSDYVMSWXRQAPGKGLEWVSATSGSGGSIYYADSVKGRFTISRDNSKNTLYLQMNSLRAEDTAVYYCAKDGPSGILTGPPPRVYFYYYYMAVWGIGTTVTVSS

SEQ ID NO: 254 - protein, 114 aa, synthetic construct
  REGION 1..114: note = light chain S.11.1.E9_L
QSALTQPASVSGSPGQSITISCTGSSSDVGSYNLVSWYQQHPGKAPKLMIYEVSKRPSGVSNRFSGSKSGNTASLTISGLQAEDEADYYCCSYAGSNTYVAFGGGTRLTVLGQP

SEQ ID NO: 255 - protein, 129 aa, synthetic construct
  REGION 1..129: note = heavy chain S.11.2.E3
EVQLLESGGGLVQPGGSLRLSCAASGFPFITYAMSWVRQAPGKGPEWVSGISSRGGKTYYADSVKGRFTISRDNDGNILSLQMNSLRAEDTAVYYCAKALLRSSGSYDGNYFYFYMDVWGKGTTVTVSS

SEQ ID NO: 256 - protein, 110 aa, synthetic construct
  REGION 1..110: note = light chain S.11.2.E3_L
QSALTQPASVSGSPGQSLTISCTGTSSDIGAYNYVSWYQQYPGKAPKLIIYDADKRPSGASDRFSGSKSGNTASLTISGLQAEDEADYYCNSYTTANTGVFGGGTKLTVL

SEQ ID NO: 257 - protein, 129 aa, synthetic construct
  REGION 1..129: note = heavy chain S.11.2.H4
EVQLVESGGGLVKPGGSLRLSCAASGFTLNTYGMNWVRQAPGKGLEWVSSISGRSNFIYYADSLRGRFTISRDNAKNSLYLQMNSLRAEDTAVYYCARDFPPETSRRFDWLLADGLDVWGQGTTVTVSS

SEQ ID NO: 258 - protein, 109 aa, synthetic construct
  REGION 1..109: note = light chain S.11.2.H4_L
QSALTQPPSASGSPGQSVTISCTGTSSDIGAYNYVSWYQQHPGKAPKFLIYGVTQRPSGVPDRFSGSKSGNTASLTVSGLQAEDEADYYCSSYAGNKVIFGGGTKLTVL

SEQ ID NO: 259 - protein, 119 aa, synthetic construct
  REGION 1..119: note = heavy chain S.11.3.A2
QVQLVESGGGVVQPGRSLRLSCAASGFTFSNYGMHWVRQAPGKGLEWVAVMSYDGSHKYYADSVKGRFTISRDNSKNTLYLQMNSLRGDDTAVYYCARDYGDYGAFDIWGQGTMVTVSS

SEQ ID NO: 260 - protein, 113 aa, synthetic construct
  REGION 1..113: note = light chain S.11.3.A2_K
DIVMTQSPDSLAVSLGERATINCKSSQSVLYSSNNKNYLAWYQQKPGQPPKLLIYWASTRESGVPDRFSGSGSGTDFTLTISSLQAEDVAVYYCHQYHTPPLTFAGGTKVEIK

SEQ ID NO: 261 - protein, 134 aa, synthetic construct
  REGION 1..134: note = heavy chain S.11.3.E11
EVQLVEPRWVLSQVQLQQSGPGLVKPSETLSLTCTVSGGSISSYYWSWIRQPPGKGLEWIGYIYYTGSTNYNPSLKSRVTIAVDTSKNQFSLKLSSVTAADTAVYYCATYYYDSSGWDYGLDVWGLGTTVTVSS

SEQ ID NO: 262 - protein, 109 aa, synthetic construct
  REGION 1..109: note = light chain S.11.3.E11_K
DIQMTQSPSSLSASVGDRVTITCRTSQRISSFLNWYQQRPGKAPKLLIYGASTLQSGVPSRFSGSGSATDFTLTISSLQPEDFATYYCQRSYGTPPALTFGGGTKVEIK

SEQ ID NO: 263 - protein, 119 aa, synthetic construct
  REGION 1..119: note = heavy chain S.11.3.F2
EVQLVESGGGLIQPGGSLRLSCGVSGFTFSQYWMNWVRQVPGKGLVWVARVSSDGSSATYADSVKGRFTISRDNAKNTLYLQMESLRVEETAVYYCARSAYLRGWFDPWGQGTLVTVSS

SEQ ID NO: 264 - protein, 111 aa, synthetic construct
  REGION 1..111: note = light chain S.11.3.F2_L
NFMLTQPHSVSESPGKTVTITCTGSSGSVANNYVQWYQQRPGSAPTLVIFEDSHRPSGVPDRFSASVDISSNSASLTISGLKTEDEADYYCQSLDSSVHVVFGGGTRLTVL

SEQ ID NO: 265 - protein, 123 aa, synthetic construct
  REGION 1..123: note = heavy chain S.11.3.F9
QVQLVESGGGVVQPGRSLRLSCAASGFPFLTYAMHWVRQAPGKGLEWVAGISSDGDTKSYADSVKGRSTISRDNYASTLYLQIDSLTTEDTAVYYCARTSGRGSNDRARFDPWGQGTLVTVSS

SEQ ID NO: 266 - protein, 111 aa, synthetic construct
  REGION 1..111: note = light chain S.11.3.F9_K
DIVMTQSPVSLPVTPGEPATISCRSSQSLLDSNGHNYLDWYLQKPGQSPQLLIYLGSTRASGVPDRFSGSGSGTDFTLKISRVEAEDVGVYYCMQALQTFTFGPGTKVDIK

SEQ ID NO: 267 - protein, 124 aa, synthetic construct
  REGION 1..124: note = heavy chain S.11.4.D10
QVQLQESGPGLVKPSETLSLTCTVSGYSIRSGYYWGWIRQPPGKGLEWLGSIHQSGNTSYNPSLKRRVTMSVDTSKNQFSLKLSSVTAADTAVYYCARIMQGRIVVLITYMDYWGQGTLVTVSS

SEQ ID NO: 268 - protein, 111 aa, synthetic construct
  REGION 1..111: note = light chain S.11.4.D10_L
  SITE 21: note = misc_feature - Xaa can be any naturally occurring amino acid
  SITE 80: note = misc_feature - Xaa can be any naturally occurring amino acid
QSVLTQPPSASGTPGQRVTIXCSGSSSNIGRNAVDWYQQVPGTAPRLLIYSNYQRPSGVPARFSGSKSGTSASLAISGLXSEDEADYYCAAWDDSLDGQVVFGGGTKLTVL

SEQ ID NO: 269 - protein, 118 aa, synthetic construct
  REGION 1..118: note = heavy chain S.11.4.F10
EVQLVETGGGLIQPGGSRRLSCAASGITVSSNYMNWVRQAPGKGLEWVAVIYSGGSTFYADSVKGRFTISRDNSKNTLYLQINSLRADDTAVYYCARGVWDDAFDIWGQGTMVTVSSA

SEQ ID NO: 270 - protein, 109 aa, synthetic construct
  REGION 1..109: note = light chain S.11.4.F10_K
DIQLTQSPSFLSASVGDRVTITCRASQGISHYLAWYQQKPGKAPKLLIYSASTLQSGVPSRFSGSGSGTEFTLTISSLQPEDFATYYCQRLNSSPSIFTFGPGTKVDIK

SEQ ID NO: 271 - protein, 119 aa, synthetic construct
  REGION 1..119: note = heavy chain S.11.4.G6
QVQLVESGGGVVQPGRSLRLSCVASGFTFSNYGMHWVRQAPGKGLEWVAVISYDGSMIYFADSVKGRSTIPRDNSKNTLYLQMNNLRPEDTAVYYCARDYGDYAALDFWGQGTMVTVSS

SEQ ID NO: 272 - protein, 113 aa, synthetic construct
  REGION 1..113: note = light chain S.11.4.G6_K
DIVMTQSPDSLAVSLGERATINCKSSQSVLFSSTNKNNLAWYQQKPGQPPTLLIYWASARQSGVPDRFSGSGSGTDFTLTITGLQAEDVAVYYCQQYHSPPLTFGGGTKVEIK

SEQ ID NO: 273 - protein, 121 aa, synthetic construct
  REGION 1..121: note = heavy chain S.11.6.H11
QVQLQESGPGLVKPSETLSLTCTVSGGSIISSAIWWNWVRQPPGKGLEWIGEVYHSGSTNYNPSLKSRVILSVDKSKNQFSLKLTSLTAADTAVYYCASKLYDYYIRYDSWGQGTLVTVSS

SEQ ID NO: 274 - protein, 108 aa, synthetic construct
  REGION 1..108: note = light chain S.11.6.H11_K
EIVLTQSPGTLSLSPGETGTLSCRASQSLSSNYVAWLQQKPGQAPRLLIYATSTRATGIPVRFSGSGSGTDFTLTVSRLEPEDFAVYYCQQYASSPVTFGAGTKVEIK

SEQ ID NO: 275 - protein, 124 aa, synthetic construct
  REGION 1..124: note = heavy chain S.11.7.A12
QVQLQESGPGLVKPSETLSLACAVSGYSISSGYYWAWLRQPPGKGLEWIGSIHQSGDTSYSPSLKSRVAISIDKSKNQFSLKLSSVTAADTAVYYCARVMQGRIVVLIAYIDYWGQGTLVTVSS

SEQ ID NO: 276 - protein, 111 aa, synthetic construct
  REGION 1..111: note = light chain S.11.7.A12_L
QSVLTQPPSASGTPGQRVTISCSGSSSNIGPNAVDWYQQLPGTAPKLLIYSNNQRPSGVPARFSGSKSGTSASLAISGLQSEDEADYYCAAWDDSLGGQVVFGGGTKLTVL

SEQ ID NO: 277 - protein, 118 aa, synthetic construct
  REGION 1..118: note = heavy chain S.11.7.A8
EVQLVESGGGLIQPGGSLRLSCAVSDLIVGDSYMTWVRQAPGKGLEWVSVIYRGGNVYHADSVKGRFTVTRDRATNTLFLHMNSLKAEDTAVYYCARRQSTSWSLDYWGQGTLVTVSS

SEQ ID NO: 278 - protein, 121 aa, synthetic construct
  REGION 1..121: note = light chain 11.7.A8_L
QSALTQPPSASGSPGQSVTISCTGTSSDVGGYKYVSWYQQRPGRAPKLIISDVTERPSGVPDRFSGSKSGNTASLTVSGLQAEDEADYYCSSYAGSNNLVFGGGTKLTVLGQPKAAPSVTL

SEQ ID NO: 279 - protein, 123 aa, synthetic construct
  REGION 1..123: note = heavy chain S.11.7.G6
  SITE 122: note = misc_feature - Xaa can be any naturally occurring amino acid
QVQLQESGPGLVKPSETLSLTCTVSGGSVSGGTYYWSWIRQHPGKGLEWIGNIYFYGSTYYNPSVGTRITLSLDTSKNHIYLRLTSVTAADTAVYYCARSYTGYQSDDALDIWGQGTMVTVXS

SEQ ID NO: 280 - protein, 106 aa, synthetic construct
  REGION 1..106: note = light chain S.11.7.G6_K
IQMTQSPSSLSASEGDRVTITCRASQDIGSDLGWYRQKPGKAPKRLIYAASSLQSGVPSRFSGSGSGTEFTLTISSLQPEDFATYYCLQHNSYPLTFGGGTKVEIK

SEQ ID NO: 281 - protein, 123 aa, synthetic construct
  REGION 1..123: note = heavy chain S.11.8.B12
QVQLVESGGGVVQPGRSLRLSCAASGFGITTYTMNWVRQAPGMGLEWVASISSDGSNTYHADSVKGRFTVSRDNYMNTLYLQLNSPRSEDTAVYYCARTSGRGSADRGRFDPWGQGTLVTVSS

SEQ ID NO: 282 - protein, 111 aa, synthetic construct
  REGION 1..111: note = light chain S.11.8.B12_K
DIVMTQSPLSLPVIPGEPASISCRSSQSLLGSNGHSYLDWYLQKPGQSPQLLIYLGSNRASGVPDRFSGSGSGTDFTLKISRVEAEDVGVYYCMQALESFTFGPGTKVDIK

SEQ ID NO: 283 - protein, 131 aa, synthetic construct
  REGION 1..131: note = heavy chain S.11.8.B2
QVQLVQSGAELKKPGASVEVSCKASGYTFTNSYIHWVRQAPGQGLEWMGIINPSGGSTSYAQKFQGRVTMTRDTSTPTVYMELSSLSSEDTAVYYCARDMGRNYDILTDYESFYYHAMDVWGQGTTVTVSS

SEQ ID NO: 284 - protein, 119 aa, synthetic construct
  REGION 1..119: note = light chain S.11.8.B2_L
SYELTQPPSVSVAPGKTASITCGGNNIGSKSVHWYQRKPGQAPVLVVYDDSDRPSGIPERFSGSKSGNTATLTISRVDAGDEADYYCQVWDSSSDPVVFGGGTKLTVLGQPKAAPSVTL

SEQ ID NO: 285 - protein, 117 aa, synthetic construct
  REGION 1..117: note = heavy chain S.11.8.C3
EVQLVETGGGLIQPGGSLRLSCAASGVTVSSNYMSWVRQAPGKGLDWVSVIYPGGTTNYADSVKGRFTISRDNSKNTLHLQMDSLRAEDTAVYYCARDFFEGAMDVWGQGTTVTVSS

SEQ ID NO: 286 - protein, 108 aa, synthetic construct
  REGION 1..108: note = light chain S.11.8.C3_K
DIQLTQSPSFLSASVGDRVTITCRASQGISSYLAWYQQKPGRAPKLLIYAASTLQSGVPSRFSGSGSGTEFTLTISSLQPEDFATYYCQQLNSYPRGTFGGGTKVEIK

SEQ ID NO: 287 - protein, 122 aa, synthetic construct
  REGION 1..122: note = heavy chain S.11.8.D2
QVQLQESGPGLVKPSETLSLTCAVSGGAVSGSNWWSWVRQPPGKGLEWIGEVYHSGNTNYNPSLKRRVVISVDRSKNQFSLHLTSLTAADTAVYFCARGPILGGGHYYLDVWGSRTTVTVSS

SEQ ID NO: 288 - protein, 111 aa, synthetic construct
  REGION 1..111: note = light chain S.11.8.D2_L
QSALTQPASVSGSPGQSITISCTGTSSDVGSYNLVSWYQQHPGKAPKLMIFQVAKRPSGVSQRFSGSKSGNTASLTISGLQAEDEADYYCCSYAGSDTYLLFGGGTKLTVL

SEQ ID NO: 289 - protein, 127 aa, synthetic construct
  REGION 1..127: note = heavy chain S.11.8.D9
EVQLVQSAAEVRKPGESLKISCKVSGYSFTNYWIAWVRQMPGKGLEWMGIIYPDDSDTRYSPSFQGQVTISADKAVNTAYLQWSSLKASDTAMYYCARHWRPSMAARPGYQYYMDVWGKGTTVTVSS

SEQ ID NO: 290 - protein, 103 aa, synthetic construct
  REGION 1..103: note = light chain 11.8.D9_K
DIQMTQSPSSLSASVGDRVTITCQASQDIDIYLNWYQQKPRKAPKLLIFDASNLETGVPSRFSGSGSGTHFTFTISSLQPEDIATYYCQQYDNLPLTFGGGTK

SEQ ID NO: 291 - protein, 127 aa, synthetic construct
  REGION 1..127: note = heavy chain S.11.8.G11
QVQLVQSGAEVKKPASSVKVSCKASGGTFNIYAITWVRQVPGQGLEWMGEIIPISNSPTYAQKFQGRILITADESSSTAFMELSSLSSEDTAVYCCARRGRFYYDSSGSYYTYFDYWGQGTLVTVSS

SEQ ID NO: 292 - protein, 106 aa, synthetic construct
  REGION 1..106: note = light chain S.11.8.G11_K
DIQMTQSPSSLSASVGDRVTITCRASQSINNYLNWYQHKPGKAPKLLIYAASSLHSGVPSRFSGSGSGTDFTLTISSLQPEDFATYYCQQSYSTPAFGQGTKVEIK

SEQ ID NO: 293 - protein, 129 aa, synthetic construct
  REGION 1..129: note = heavy chain S.11.8.G8
EVQLLEAGGGLVQPGGSLTLSCEASGFPFITYAMNWVRQAPGKGPEWISAISSGGDRTFYADSVKGRFTVSRDNPGNILYLQMNSLSAEDTAVYYCAKALLRGSGSFHGNYYYYYMDVWGKGTTVTVSS

SEQ ID NO: 294 - protein, 110 aa, synthetic construct
  REGION 1..110: note = light chain S.11.8.G8_L
QSALTQPASVSGSPGQSITISCTGTSTDVGGYDYVSWYQQHPGKAPKLIIYDVTKRPSGVSDRFSGSKSGNTASLTISGLQADDEAHFYCTSYTATTVALFGGGTKLTVL

SEQ ID NO: 295 - protein, 123 aa, synthetic construct
  REGION 1..123: note = heavy chain S.3.1.A6
QVQLVESGGGVVQPGRSLRLSCAASGFTFSSYGMHWVRQAPGKGLEWVAVIWYDGSNKYYADSVKGRFTISRDNSKNTLYLQMNSLRAEDTAVYYCAREGYSSSWYRTRFDYWGQGTLVTVSS

SEQ ID NO: 296 - protein, 105 aa, synthetic construct
  REGION 1..105: note = light chain S.3.1.A6_K
DIQMTQSPSSLSASVGDRVTITCRASQSISSYLNWYQQKPGKAPKLLIYAASSLQSGVPSRFSGSGSGTDFTLTISSLQPEDFATYYCQQSYSYTFGQGTKLEIK

SEQ ID NO: 297 - protein, 114 aa, synthetic construct
  REGION 1..114: note = heavy chain S.3.2.F6
  SITE 2: note = misc_feature - Xaa can be any naturally occurring amino acid
  SITE 109: note = misc_feature - Xaa can be any naturally occurring amino acid
EXGAEVKKPGESLKISCKGSGYSFTSYWIGWVRQMPGKGLEWMGIIYPGDSDTRYSPSFQGQVTISADKSISTAYLQWSSLKASDTAMYYCARLRGVIMPQYGMDVWGXGTTVT

SEQ ID NO: 298 - protein, 97 aa, synthetic construct
  REGION 1..97: note = light chain S.3.2.F6_K
  SITE 84: note = misc_feature - Xaa can be any naturally occurring amino acid
  SITE 90: note = misc_feature - Xaa can be any naturally occurring amino acid
  SITE 93: note = misc_feature - Xaa can be any naturally occurring amino acid
  SITE 97: note = misc_feature - Xaa can be any naturally occurring amino acid
LSASVGDRVTITCRASQSISSWLAWYQQKPGKAPKLLIYKASSLESGVPSRFSGSGSGTEFTLTISSLQPDDFATYYCQQYNSXSRTFGXGTXLEIX

SEQ ID NO: 299 - protein, 118 aa, synthetic construct
  REGION 1..118: note = heavy chain S.3.3.A4
EVQLVETGGGVIQPGVSLRLSCAVSGFNVGRTYMSWVRQTPGRGLEWVAVIYTDATTYYPDSLRGRFSISRDNWKNTVSLQMSSLRGEDTAIYYCAGGLKYPNTFDFWGQGTLVTVSS

SEQ ID NO: 300 - protein, 111 aa, synthetic construct
  REGION 1..111: note = light chain S.3.3.A4_K
DIVMTQSPLSLPVTPGEPASISCRSSQSLLNNDGNIYLDWYLQKPGQSPQLLIYLASIRASGVPDRFSGSGSGTDFTLKISRVEAEDVGLYYCMQGQYAPTFGQGTRLEIK

SEQ ID NO: 301 - protein, 118 aa, synthetic construct
  REGION 1..118: note = heavy chain S.3.3.E10
EVQLVETGGGVIQPGVSPRLSCAASGFTVGSSYMSWVRQAPGRGLEWVSVIYKDGAPYYADSVRGRFTISRDDSTNTVSLQMTRLRAEDTAMYFCARGLRLPNTFDQWGQGTLVTVSS

SEQ ID NO: 302 - protein, 111 aa, synthetic construct; identical to SEQ ID NO: 300
  REGION 1..111: note = light chain S.3.3.A4 _K

SEQ ID NO: 303 - protein, 124 aa, synthetic construct
  REGION 1..124: note = heavy chain S.3.3.G8
QVQLQQWGAGLLKPSETLSLTCAVYSESFRGYYWSWIRQPPGKRLEWIGEINHSGRTNYNPSLKSRAAISVDTSRNQFSLILSSVTAADTAVYYCARGYGLGTYTWGWAPFDYWGQGSLVTVSS

SEQ ID NO: 304 - protein, 108 aa, synthetic construct
  REGION 1..108: note = light chain S.3.3.G8_K
EIVLTQSPGTLSLSPGERATLSCTASQSVSSSYLAWYQQKPGQAPRLLTYGASSRATAIPHRFSGGGSGTDFTLTISRLEPEDFAVYYCQQYGSAPHTFGQGTKVEIK

SEQ ID NO: 305 - protein, 121 aa, synthetic construct
  REGION 1..121: note = heavy chain S.5.1.A5
QVQLQQWGAGLLKPSETLSLSCAVYGGSFSGYYWSWIRQPPGKGLEWIGEINHSGSTNYNPSLKSRVTISVDTSKNQFSLQLNSVSPEDTAVYYCAMTTKNSEGYWYFDLWGRGTLVTVSS

SEQ ID NO: 306 - protein, 108 aa, synthetic construct
  REGION 1..108: note = light chain S.5.1.A5_K
EIVLTQSPATLSLSPGERATLSCRASQSVSSYLAWYQQKPGQAPRLLIYDASNRATGIPTRFSGSGSGTDFTLTISNLEPGDFAVYYCQQRSDWPPYTFGQGTKLEIK

SEQ ID NO: 307 - protein, 120 aa, synthetic construct
  REGION 1..120: note = heavy chain S.5.1.B8
QVQLVESGGGVVQPGRSLRLSCVASGFTFSSYAMHWVRQAPGKGLEWVAVISYDGGDRYYTDSVKGRFTISRDNSKSTLYLQMNSLRAEDTAVYYCAKDLSRGYDSDDYWGQGTLVTVSS

SEQ ID NO: 308 - protein, 110 aa, synthetic construct
  REGION 1..110: note = light chain S.5.1.B8_L
QSVLTQPPSASGTPGQRVTISCSGSSSNIGSNYVYWYQQLPGTAPQLLIYTNNQRPSGIPDRFSGSKSGTSASLAISGLRSEDEADYYCATWDDSLSGWVFGGGTKLTVL

SEQ ID NO: 309 - protein, 125 aa, synthetic construct
  REGION 1..125: note = heavy chain S.6.1.F8
EVQLVESGGGVVRPGGSLRLSCAASGFTFDDYGMSWVRQAPGKGLEWVSGINWNGGSTGYADSVKGRFTISRDNAKNSLYLQMNSLRAEDTALYYCARDPSIATTADYYYGMDVWGQGTTVTVSS

SEQ ID NO: 310 - protein, 106 aa, synthetic construct
  REGION 1..106: note = light chain S.5.1.A11_K
MTQSPASLSASVGDRVTITCRASQGIRNDLGWYQQKPGKAPKRLIYAASSLQSGVPSRFSGSGSGTEFTLTISSLQPEDFATYYCLQHNSYPSTWTFGQGTKVEIK

SEQ ID NO: 311 - protein, 119 aa, synthetic construct
  REGION 1..119: note = heavy chain S.6.1.H8
QVQLVESGGGVVQPGRSLRLSCAASGFTFKTYGMHWVRQAPGKGLEWVAVISYDEKTTYYADSVKGRFTISRDNSKNTLYLQIKNSRREDTAVYLCAKGGSAAAVLDYWGQGTLVTVSS

SEQ ID NO: 312 - protein, 113 aa, synthetic construct
  REGION 1..113: note = light chain S.6.1.H8_K
DIVMTQSPDSLTVPLGERATISCKSSQSLFYRSNSKNYLAWYQQKAGQPPTPLIYWASTRESGVPDRFSGSGSGTDFTLTISSLQAEDVAVYYCQQYYRTPLTFGGGTKVEIK

SEQ ID NO: 313 - protein, 126 aa, synthetic construct
  REGION 1..126: note = heavy chain S.7.11.B7
QVQLVQSGAEVKKPGASVNVSCKASGYTFTSYGISWVRQAPGQGLEWMGWISAYNGNTNYAQKIQGRVTMTTDTSTSTAYMELRSLRSDDTAVYYCARVSRSVWFGEARKSAMDVWGQGTTVTVSS

SEQ ID NO: 314 - protein, 107 aa, synthetic construct
  REGION 1..107: note = light chain S.7.11.B7_K
DIQMTQSPSTLSASVGDRVTITCRASQSISSWLAWYQQKPGKAPKLLIYKASNLQDGVPSRFSGSGSGTEFTLTISSLQPDDFATYYCQQCNTYPWTFGQGTKVEIK

SEQ ID NO: 315 - protein, 126 aa, synthetic construct
  REGION 1..126: note = heavy chain S.8.2.B6
QVQLVQSGPEVRKPGASVKVSCKASGYIFSSYAISWVRQAPGQGLEWMGFISTYNGDAKYAQKYQGRVTMTIDTSTSTAYMELRSLRSDDTAVYYCARDLTGEEYYYDSSDAFDIWGQGTMVTVSS

SEQ ID NO: 316 - protein, 107 aa, synthetic construct
  REGION 1..107: note = light chain S.8.2.B6_K
DIQMTQSPSTLSASEGDRVTITCRASQSISSWLAWYQQKPGKAPKLLIYKASSLESGVPSRFSGSGSGTEFTLTISSLQPDDFATYYCQQYHSYSLTFGGGTKVEIK

SEQ ID NO: 317 - protein, 124 aa, synthetic construct
  REGION 1..124: note = heavy chain S.8.2.E3
EVQLLESGGGLVQPGGSLRLSCAGSGFTFSSYAMTWVRQAPGKGLEWVSTISGGGGSTYYADSVKGRFTISRDNSKNTLYLQMNSLRAEDTALYYCAKGERIIILVAVTFLDYWGQGTLVTVSS

SEQ ID NO: 318 - protein, 108 aa, synthetic construct
  REGION 1..108: note = light chain S.8.2.E3_L
  SITE 5: note = misc_feature - Xaa can be any naturally occurring amino acid
QSVLXQPPSVSAAPGQKVTISCSGGSSNIGNNYVSWFQHLPGTAPKLLIYDSNKRPSGIPDRFSGSKSGTSATLGITGLQTGDEADYYCGTWDSSLSAYVFGTGTKVT

SEQ ID NO: 319 - protein, 130 aa, synthetic construct
  REGION 1..130: note = heavy chain S.8.2.F3
QVQLQESGPGLVKPSQTLSLTCSVSGGSITSGSYFWSWIRQPAGKGLEWIGRIYPTGSTNYNPSLKSRVSISVDTSKNQFSLRLSSVTAADTAVYYCARAPHRIYYYDRSGDYYDAFDIWGQGSMVTVSS

SEQ ID NO: 320 - protein, 110 aa, synthetic construct
  REGION 1..110: note = light chain S.8.2.F3_L
QSVLTQPPSASGTPGQRVTISCSGSSSNIGSNTVNWYQQLPGTAPKLLIYSNNQRPSGVPDRFSGSTSGTSASLAISGLQSEDEADYYCATWDDSLNGYVVFGGGTKLTV

SEQ ID NO: 321 - protein, 121 aa, synthetic construct
  REGION 1..121: note = heavy chain S.9.1.B2
QVQLVESGGGVVQPGRSLRLSCVASGFTFSRYGMHWVRQAPGKGLEWVAVISYDGSNKDYADSVKGRFTISRDISKNTLYLQMNSLRAEDTAVYYCAKEVGYSDYDVGDYWGQGTLVTVSS

SEQ ID NO: 322 - protein, 107 aa, synthetic construct
  REGION 1..107: note = light chain S.9.1.B2_K
DIQMTQSPSSLSTSVGDRVTITCQASQDIRNYLNWYQQKPGKAPKLLIYDASNLEIGVPSRFSGSGSGTDFTFTISSLQPEDIATYYCQQYANLPLTFGGGTKVEIK

SEQ ID NO: 323 - protein, 130 aa, synthetic construct
  REGION 1..130: note = heavy chain S.9.1.C7
QVQLQESGPGLVKPSQTLSLTCTVSGGSISSGSYYWSWIRQPAGKGLEWIGRIFPTGSTNYNPSLKSRVTISVDTSKNQFSLKLSSVTAADTAVYFCAREPFKMYYYDNSDYYYDAFDIWGQGTMVTVSS

SEQ ID NO: 324 - protein, 110 aa, synthetic construct
  REGION 1..110: note = light chain S.9.1.C7_L
QSALTQPRSVSGSPGQSVTISCTGTSSDVGGYNYVSWYQHHPGKAPKLMIYDVSKRPSGVPDRFSGSKSGNTASLTISGLQAEDEADYYCCSYAGRYTYVFGTGTKVTVL

SEQ ID NO: 325 - protein, 114 aa, synthetic construct
  REGION 1..114: note = heavy chain S.9.1.D5
EVQLVESGGGLVQPGGSLRLSCAGSGFTVSSNYMSWVRQAPGKGLEWVSVIYSGGSTKYADSVKGRFTISRDNSKNTLYLQMNSLRLEDTAVYYCARDLEGTDWGQGTLVTVSS

SEQ ID NO: 326 - protein, 107 aa, synthetic construct
  REGION 1..107: note = light chain S.9.1.D5_K
EIVMTQSPATLSVSPGERATLSCRASQSVSTNLAWYQQKPGQAPRLLIYGASTRATSIPARFSGSGSGTEFTLTISSLQSGDFAVYYCQQYNNWPRTFGQGTKVEIK

SEQ ID NO: 327 - protein, 123 aa, synthetic construct
  REGION 1..123: note = heavy chain S.9.1.H9
QLQLQESGPGLVKPSETLSLTCTVSGDSISSSSYYWGWIRQPPGKGLEWIGSIFYSGSTYYNPSLKSRVTISVDTSNNQFSLKLSSVTAADTAVYYCARLYDTYYYHHGMDVWGQGTTVTVSS

SEQ ID NO: 328 - protein, 106 aa, synthetic construct
  REGION 1..106: note = light chain S.9.1.H9_K
IQMTQSPSSLSASVGDRVTITCRASQDIRNDLGWYQQKPGKAPKRLIYAASSLQSGVPSRFSGSGSGTEFTLTITSLQPEDFATYSCLQHNSYPLTFGGGTKVEIK

SEQ ID NO: 329 - protein, 128 aa, synthetic construct
  REGION 1..128: note = heavy chain S.9.2.E3
QVQLVQSGAEVKKPGASVKVSCKVSGYTLTEVSIHWVRQAPGKGLEWMGGFDPEDAETIYAQKFQGRVTMTEDTSTDTAYMELSSLRSDDTAVYYCAAGVAVTGTPLAYSYYYGMDVWGQGTTVTVSS

SEQ ID NO: 330 - protein, 104 aa, synthetic construct
  REGION 1..104: note = light chain S.9.2.E3_K
MTQSPATLSVSPEQRATLSCRASQSVSSNLAWYQQKPGRAPRLLIYGTSTRATGIPARFSGSGSGTEFTLTISSLQSEDFAVYYCQQYNNWPLTFGGGTKVEIK

SEQ ID NO: 331 - protein, 124 aa, synthetic construct
  REGION 1..124: note = heavy chain S.9.2.F3
  SITE 10: note = misc_feature - Xaa can be any naturally occurring amino acid
EVQLLESGGXLVQPGGSLRLSCAASGFTFSNYVMNWVRQAPGKGLEWVSTISGSGSTTYYADSVKGRFTISRDNSKNTLYLQMNSLRAEDTAVYYCAKGERIIMIVVVTFFDYWGQGTLVTVSS

SEQ ID NO: 332 - protein, 109 aa, synthetic construct
  REGION 1..109: note = light chain S.9.2.F3_L
QSVLTQPPSVSAAPGQKVTISCSGSSSNIGNNYVSWFQQLPGTAPKLLIYDNNKRPSGIPDRFSGSKSGTSATLGITGLQTGDEADYYCGTWDSSLSAVVFGGGTKLTV

SEQ ID NO: 333 - protein, 124 aa, synthetic construct
  REGION 1..124: note = heavy chain S.9.2.G1
EVQLLESGGGLVQPGGSLRLSCAASGLTFSSYAMSWVRQAPGKGLEWVSSISGGGGSTYYADSVKGRFTISGDNSKNTLFLQMNSLRAEDTAVYYCAKNERIITMVVITLFDYWGQGTLVTVSS

SEQ ID NO: 334 - protein, 109 aa, synthetic construct
  REGION 1..109: note = light chain S.9.2.G1_L
QSVLTQPPSVSAAPGQKVTISCSGSSSNIGKNYVSWYQRLPGTAPKLLIYDNNKRPSGIPDRFSGSKSGTSATLGITGLQPGDEADYYCGTWDRSLSAWVFGGGTKLTV

SEQ ID NO: 335 - protein, 127 aa, synthetic construct
  REGION 1..127: note = heavy chain S.9.3.D5
EVQLVESGGGLVKPGGSLRLSCAASGFTFSSYSMNWVRQAPGKGLEWVSSISSSNSYIYYADSVKGRFTISRDNAKNSLYLQMNSLRAEDTAVYYCARWKLPYYDSSGYYPEAFDIWGQGTMVTVSS

SEQ ID NO: 336 - protein, 108 aa, synthetic construct
  REGION 1..108: note = light chain S.9.3.D5_K
EIVMTQSPATLSVSPGERATLSCRASQSVSNNLAWYQQKPGQAPRLLIYGASTRATGFPARFSGSGSGTEFTLTISSLQSEDFAVYYCQQYYNWPPWTFGQGTKVEIK

SEQ ID NO: 337 - protein, 132 aa, synthetic construct
  REGION 1..132: note = heavy chain S.9.3.F7
QVQLQESGPGLVKPSQTLSLTCTVSGDSISSGDYYWSWIRQPPGKGLEWIGYIYYTGITYYNPSLKSRVTISVDTSKNQFSLKLSSVTAADTAMYYCVRARVVPAAISDAQNYYYYYGMDVWGQGTTVTVSS

SEQ ID NO: 338 - protein, 112 aa, synthetic construct
  REGION 1..112: note = light chain S.9.3.F7_K
DIVMTQSPLSLPVTPGEPASISCRSSQSLLHSNGYNYLDWYLQKPGQSPQLLIYLGSNRASGVPDRFSGSGSGTDFTLEISRVEAEDVGVYYCMQALQTPFTFGQGTRLEIK

SEQ ID NO: 339 - protein, 125 aa, synthetic construct
  REGION 1..125: note = heavy chain S.9.3.G1
EVQLVESGGGLVKPGGSLRLSCAASGFAFSNAWMNWVRQAPGKGLEWVGRIKSETDGGTTDYAAPVKGRFTISRDDSKNTLYLQMNSLKTEDTAVYYCVTVSPGYNYGYEDFDHWGQGTLVTVSS

SEQ ID NO: 340 - protein, 109 aa, synthetic construct
  REGION 1..109: note = light chain S.9.3.G1_K
EIVLTQSPGTLSLSPGERATLSCRASQSFSRSYLAWYHQKPGQAPRLLIYGASSRATGIPDRFSGSGSGTDFTLTISRLEPEDFAVYYCQHYGSSPPITFGQGTRLEIK

SEQ ID NO: 341 - protein, 128 aa, synthetic construct
  REGION 1..128: note = heavy chain S.9.3.H10
QVQLVQSGSELKKPGASVKVSCKASGYTFTTYAMNWVRQAPGQGLEWMGWINTNTGNPMYAQGFRGRYVFSLDTSVSTAYLQISSLKAEDTAVYYCARDDVVSVVGTAHYYYYGMDVWGQGTTVTVSS

SEQ ID NO: 342 - protein, 111 aa, synthetic construct
  REGION 1..111: note = light chain S.9.3.H10_L
  SITE 17: note = misc_feature - Xaa can be any naturally occurring amino acid
QSVLTQPPSASATPGQXVTISCSGSSSNIGSNFVYWYQQLPGTAPKLLIYSNDQRPSGVPDRFSGSKSGTSASLAISGLRSEDEADYYCAAWDDSLRGLWVFGGGTKLTVL

SEQ ID NO: 343 - protein, 123 aa, synthetic construct
  REGION 1..123: note = heavy chain S.9.4.B6
QVQLQESGPGLVKPSGTLSLTCAVSGASISSGNWWSWVRQPPGKGLEWIGEVYHSGNTNYNPSLKSRVTMSVDKSKNQFSLKLSSVTAADTAVYYCAPRYCSSTSCPNWFDPWGQGTLVTVSS

SEQ ID NO: 344 - protein, 110 aa, synthetic construct
  REGION 1..110: note = light chain S.9.4.B6_L
QSALTQPASVSGSPGQSITISCTGTSSDVGSYNVVSWYQQHPGKAPKVMIYEASKRPSGVSNRFSGSKSGNTASLTISGLQAEDEADYYCCSYAGSSTWVFGGGTKLTVL

SEQ ID NO: 345 - protein, 129 aa, synthetic construct
  REGION 1..129: note = heavy chain S.9.4.B8
QVQLQESGPGLVKPSQTLSLTCTVSGGSISSGSYYWSWIRQPAGKGLELIGRIYTSGGTNYNPSLKSRVTISVDRSKNQFSLKLSSVTAADTAVYYCARYTHRAYYYDSSSYYDAFDIWGQGTMVTVSS

SEQ ID NO: 346 - protein, 110 aa, synthetic construct
  REGION 1..110: note = light chain S.9.4.B8_L
  SITE 2: note = misc_feature - Xaa can be any naturally occurring amino acid
QXALTQPPSASGSRGQSVTISCTGTSSDVGGYNYVSWYQQHPGKAPKLMIYEVSKRPSGVPDRFFGSKSGNTASLTVSGLQAEDEADYYCSSYGGSNNYVFGTGTKVTVL

SEQ ID NO: 347 - protein, 133 aa, synthetic construct
  REGION 1..133: note = heavy chain S.9.4.C4
QVQLQESGPGLVKPSQTLSLTCTVSGDSISSGDYYWTWIRQPPGKGLEWIGYIYYSGITYYNPSLKSRVTISVDTSRNQFSLKLSSVTAADTAMYYCARIVVVPAAIAAERRDYYYYYGMDVWGQGTTVTVSS

SEQ ID NO: 348 - protein, 112 aa, synthetic construct
  REGION 1..112: note = light chain S.9.4.C4_K
  SITE 2: note = misc_feature - Xaa can be any naturally occurring amino acid
  SITE 23: note = misc_feature - Xaa can be any naturally occurring amino acid
  SITE 33: note = misc_feature - Xaa can be any naturally occurring amino acid
DXVMTQSPLSPPVTPGEPASISXRSSQSLLHSXGYNYLDWYLQKPGQSPQLLIYLGSNRASGVPDRFSGSGSGTDFTLKISRVEAEDVGVYYCMQALQTPFTFGPGTKVDIK

SEQ ID NO: 349 - protein, 117 aa, synthetic construct
  REGION 1..117: note = heavy chain S.9.4.E1
QVQLVESGGGVVQPGRSLRLSCAASGFTFSSYAMHWVRQAPGKGLEWVALISYDGSNKYYADSVKGRFTISRDNSKNTLYLQMNSLRAEDTAVYYCARDSGSQLDYWGQGTLVTVSS

SEQ ID NO: 350 - protein, 106 aa, synthetic construct
  REGION 1..106: note = light chain S.9.4.E1_L
  SITE 27: note = misc_feature - Xaa can be any naturally occurring amino acid
SYELTQAPSVSVSPGQTASITCSGDKXGDKYACWYQQKPGQSPVLVIYQDSKRPSGIPERFSGSNSGNTATLTISGTQAMDEADYYCQAWDSRTVVFGGGTKLTVL

SEQ ID NO: 351 - protein, 123 aa, synthetic construct
  REGION 1..123: note = heavy chain S.9.5.B2
QVQLQESGPGLVKPSGTLSLTCTVSGDSISSSNWWSWVRQPPGKGLEWIGEIYHSGNTNYNPSLKSRVTISVDKAKNQFSLKLTSVTATDTAVYYCASRYCSSTACPNWFDPWGQGTLVTVSS

SEQ ID NO: 352 - protein, 111 aa, synthetic construct
  REGION 1..111: note = light chain S.9.5.B2_L
QSALTQPASVSGSPGQSITISCTGTSSDVGSYNLVSWYQQHPDKAPKLMIYEVNKRPSGVSNRFSGSKSGNTASLTISGLRAEDEADYYCCSYAGSSTFVVLGGGTKLTVL

SEQ ID NO: 353 - protein, 123 aa, synthetic construct
  REGION 1..123: note = heavy chain S.9.5.B8
QVQLQESGPGLVKPSGTLSLTCAVSGGSISSGDWWSWVRQPPGKGLEWIGEIYHSGNTNYSPSLKSRVTISVDNSKNQFSLKLNSVTAADTAVYYCARRYCSSTTCPNWFDPWGQGTLVTVSS

SEQ ID NO: 354 - protein, 107 aa, synthetic construct
  REGION 1..107: note = light chain S.9.5.B8_K
DIQMTQSPSSLSASVGDRVTITCRASQVISNSLAWYQQKPGKAPKFLIYAASTLESGVPSRFSGSGSGTDFTLTISSLQPEDFATYYCQQYYDAPRTFGQGTKVEIK

SEQ ID NO: 355 - protein, 128 aa, synthetic construct
  REGION 1..128: note = heavy chain S.9.5.C6
QVQLVQSGSELKKPGASVKVSCKASGYSFSSYAMNWVRQAPGQGLEWMGWINTNTGKPTYAQDFTGRFVFSLDTSVNTAYLQISSLKAEDTAVYYCARVQGVGVVAESYYYYYAMDVWGQGTTVTVSS

SEQ ID NO: 356 - protein, 109 aa, synthetic construct
  REGION 1..109: note = light chain S.9.5.C6_K
EIVLTQSPATLSLSPGERATLSCRASQNISSFLGWYQQKPGQAPRLLIYDASNRATGIPARFSGSGSGTDFTLTISSLETEDFAIYYCQQRSKWPPEGTFGQGTKLEIK

SEQ ID NO: 357 - protein, 121 aa, synthetic construct
  REGION 1..121: note = heavy chain S.11.1.E5
EVQLVESGGGLAQPGKSLRLSCTASGFTFDDYAMHWVRQVPGKGLEWVSGISWNGDSIGYGASVKGRFTISRDNAKNSLYLQMNSLRDEDTALYYCAKGRYVDWTHAMDVWGQGTTVTVSS

SEQ ID NO: 358 - protein, 108 aa, synthetic construct; identical to SEQ ID NO: 110
  REGION 1..108: note = light chain S.11.1.E10_L

SEQ ID NO: 359 - protein, 121 aa, synthetic construct; identical to SEQ ID NO: 357
  REGION 1..121: note = heavy chain S.11.1.E5

SEQ ID NO: 360 - protein, 108 aa, synthetic construct; identical to SEQ ID NO: 130
  REGION 1..108: note = light chain S.11.7.A5_L